European Patent Application EP 4 230 649 A2, published August 23, 2023. Title: ANTIBODIES AND METHODS FOR THE DIAGNOSIS AND TREATMENT OF EPSTEIN BARR VIRUS INFECTION. Applicant: The U.S.A. as represented by the Secretary, Department of Health and Human Services. Application EP, filed April 25, 2018. The sequence listing filed with the application follows.

SEQUENCE LISTING (293 sequences)

SEQ ID NO: 1 - protein, 121 aa, Homo sapiens
QVQLQESGPGLVKPAETLSLTCTVSGGSFSSYWWGWIRQSPGKGLEWIGHISSGGNNYLNPSLKSRVTLSLDTSKNQFSLKLNSVTAADSAVYYCARAPRIVVRGRYFDQWGQGVLVTVSS

SEQ ID NO: 2 - DNA, 363 bp, Homo sapiens
  source 1..363: mol_type = genomic DNA
caggtgcagctgcaggagtcgggcccaggactggtgaagcctgcggagaccctgtccctcacctgcactgtctctggtggctctttcagcagttactggtggggctggatccgtcagtccccagggaagggactggagtggattgggcatatcagtagtggtggaaacaactaccttaatccgtccctcaagagtcgagtcaccctgtcactagacacgtccaagaaccagttctccctgaagctgaactctgtgaccgccgcggactcggccgtgtattactgtgccagagccccccgtattgttgttagaggccgatactttgaccaatggggccagggagtcctggtcaccgtctcctca

SEQ ID NO: 3 - protein, 8 aa, Homo sapiens
GGSFSSYW

SEQ ID NO: 4 - protein, 7 aa, Homo sapiens
ISSGGNN

SEQ ID NO: 5 - protein, 16 aa, Homo sapiens
APAPRIVVRGRYFDQW

SEQ ID NO: 6 - protein, 107 aa, Homo sapiens
DIQMTQSPSSLSASVGDTVTITCRASQGINIYLNWFQQRPGKAPKLLIYAATTLQSGVPSRFSGSGSGTDFTLTISSLQPEDFATYYCLQCESYPLTFGGGTKVEIK

SEQ ID NO: 7 - DNA, 321 bp, Homo sapiens
  source 1..321: mol_type = genomic DNA
gacatccagatgacccagtctccatcctccctgtctgcatctgtaggagacactgtcaccatcacttgccgggcaagtcagggtatcaatatctacctgaattggtttcagcagagaccagggaaagcccctaaactcctgatctatgctgcgaccactttacaaagtggggtcccatcaagattcagcggcagtggatctgggacagatttcactctcaccatcagcagcctgcagcctgaagatttcgcaacttattactgtctacagtgtgaaagttatccgctcactttcggcggagggaccaaggtggagatcaaa

SEQ ID NO: 8 - protein, 6 aa, Homo sapiens
QGINIY

SEQ ID NO: 9 - skipped

SEQ ID NO: 10 - protein, 9 aa, Homo sapiens
LQCESYPLT

SEQ ID NO: 11 - protein, 123 aa, Homo sapiens
QVQLQESGPGLVKPSETLSLTCTVSGGSISGAYYYWSWIRQPPGKGLDWIGYIYGSFGSAYYNPSLKSRATISKDTPKNQFSLKLSSVTAADTAVYYCARGRRLGYSNWFDVWGPGVLVTVSS

SEQ ID NO: 12 - DNA, 369 bp, Homo sapiens
  source 1..369: mol_type = genomic DNA
caggtgcaactgcaggagtcgggcccaggactggtgaagccttcggagaccctgtccctcacctgcactgtctctggtggctccatcagcggtgcttactactactggagctggattcgacagcccccggggaagggactggactggattggatatatctatggaagttttgggagtgcctactacaacccctccctcaagagtcgagccaccatttcaaaagacacgcccaagaaccagttctccctgaaactgagctctgtgaccgccgcggacacggccgtgtattactgtgcgagaggaaggcgactaggctattcgaactggttcgatgtctggggcccgggagtcctggtcaccgtctcctca

SEQ ID NO: 13 - protein, 10 aa, Homo sapiens
GGSISGAYYY

SEQ ID NO: 14 - protein, 8 aa, Homo sapiens
IYGSFGSA

SEQ ID NO: 15 - protein, 15 aa, Homo sapiens
ARGRRLGYSNWFDVW

SEQ ID NO: 16 - protein, 107 aa, Homo sapiens
DIQMTQSPSSLSASVGDKVTITCRTSQDVSSYLAWYQQKPGKAPQLLIYAASSLQSGVPSRFTGSGSGAEFTLTISSLQPEDFASYYCQQYKNLPLTFGGGTKVEIK

SEQ ID NO: 17 - DNA, 321 bp, Homo sapiens
  source 1..321: mol_type = genomic DNA
gacatccagatgacccagtctccatcttccctgtctgcatctgtaggagacaaagtcaccatcacttgtcggacaagtcaggacgttagcagttatttagcctggtatcagcagaaaccagggaaagcccctcagctcctgatctatgctgcatccagtttgcaaagtggggtcccatcaaggttcaccggcagtggatctggggcagaattcactctcaccatcagcagccttcagcctgaagattttgcatcatattactgtcaacagtataaaaatctcccgctcactttcggcggagggaccaaagtggagatcaaa

SEQ ID NO: 18 - protein, 6 aa, Homo sapiens
QDVSSY

SEQ ID NO: 19 - skipped

SEQ ID NO: 20 - protein, 9 aa, Homo sapiens
QQYKNLPLT

SEQ ID NO: 21 - protein, 129 aa, Homo sapiens
QVQLQESGPGLVKPSETLSLTCDVSGGSFSGDFYWSWIRQPPGKGLDWIGNIHGSSAGTKYKPSLKSRVTISKDTSKNQFSLKLSSVTAADTAVYYCTRGPLSRIVAGFGRGINWFDVWGPGVLVTVSS

SEQ ID NO: 22 - DNA, 387 bp, Homo sapiens
  source 1..387: mol_type = genomic DNA
caggtgcagctgcaggagtcgggcccaggactggtgaagccttcggagaccctgtccctcacctgcgatgtctctggtggctccttcagcggtgatttctactggagctggatccgccagcccccagggaagggactggactggattgggaatatccatggcagcagtgcgggcaccaaatacaagccctccctcaagagtcgagtcaccatttcaaaagacacgtccaagaaccagttctccctgaaactgagctctgtgaccgccgcggacacggccgtctattactgtacgagaggcccccttagtaggatagtagctggttttgggagggggattaactggttcgatgtctggggcccgggagtcctggtcaccgtctcctca

SEQ ID NO: 23 - protein, 9 aa, Homo sapiens
GGSFSGDFY

SEQ ID NO: 24 - protein, 8 aa, Homo sapiens
IHGSSAGT

SEQ ID NO: 25 - protein, 22 aa, Homo sapiens
TRGPLSRIVAGFGRGINWFDVW

SEQ ID NO: 26 - protein, 116 aa, Homo sapiens
QPVLTQPTSLSASPGASVRLSCTLSSGINVGSYSIFWYQQKPGSPPRYLLFYFSDSSKHQGSGVPSRFSGSKDTSANAGLLLISGLQSEDEADYYCAIWHSSASVLFGGGTRLTVL

SEQ ID NO: 27 - DNA, 348 bp, Homo sapiens
  source 1..348: mol_type = genomic DNA
cagcctgtgctgacccagccaacctccctctcagcatctccgggagcatcagtcagactcagctgcaccttgagcagtggcatcaatgttggtagttacagcatattctggtaccagcagaagccagggagtcctccccggtaccttctgttctatttctcagactcaagtaagcaccagggctctggagtccccagccgtttctctggatccaaggatacttcagccaatgcagggcttttactgatctctgggctccagtctgaagatgaggctgactattactgtgccatatggcacagcagcgcttctgtgttattcggaggagggacccggctgacagtacta

SEQ ID NO: 28 - protein, 14 aa, Homo sapiens
TLSSGINVGSYSIF

SEQ ID NO: 29 - protein, 7 aa, Homo sapiens
YFSDSSK

SEQ ID NO: 30 - protein, 10 aa, Homo sapiens
AIWHSSASVL

SEQ ID NO: 31 - protein, 120 aa, Homo sapiens
QLQLQESGPGLVKPSETLSLTCAVSGGSISGYYWSWIRQPPGKGPEWIGFIDGNTVGTNYNPSLKSRVTLSKDTSKNQFSLKVSSVTAADTAVYYCARKPLRRYFWFDVWGPGVLVTVSS

SEQ ID NO: 32 - DNA, 360 bp, Homo sapiens
  source 1..360: mol_type = genomic DNA
cagctgcagctgcaggagtcgggcccaggactggtgaagccttcggagaccctgtccctcacctgcgctgtctctggtggctccatcagcggttactactggagttggattcgccagcccccagggaagggaccggagtggattgggtttattgatggtaatactgtgggcaccaactacaacccctccctcaagagtcgagtcaccctttcaaaagacacgtccaagaatcagttctccctgaaggtgagttctgtgaccgccgcggacacggccgtgtattactgtgcgaggaagccgctacgccgttatttctggttcgatgtctggggcccgggagtcctggtcaccgtctcctca

SEQ ID NO: 33 - protein, 8 aa, Homo sapiens
GGSISGYY

SEQ ID NO: 34 - protein, 8 aa, Homo sapiens
IDGNTVGT

SEQ ID NO: 35 - protein, 14 aa, Homo sapiens
ARKPLRRYFWFDVW

SEQ ID NO: 36 - protein, 111 aa, Homo sapiens
QSVLTQPPSVSGDPGQRVTISCTGSSSNIGAGYYVYWYQQFPGTAPKLLIYQDNKRPSGVSDRFSGSKSGTSASLTITGLQPGDEADYYCSAWDSSLSAVMFGRGTRLTVL

SEQ ID NO: 37 - DNA, 333 bp, Homo sapiens
  source 1..333: mol_type = genomic DNA
cagtctgtgctgacgcagccgccctcagtgtctggggaccccgggcagagggtcaccatctcgtgcactgggagcagctccaacatcggggcgggttattatgtatactggtaccagcagttcccaggaacggcccccaaactcctcatctatcaagataataagcgaccctcaggggtttctgaccgattctctggctccaagtctggtacctcagcctccctgaccatcactgggctccagcctggggatgaggctgattattactgctcagcatgggatagcagcctgagtgctgttatgttcggaagaggcaccaggctgacagtacta

SEQ ID NO: 38 - protein, 9 aa, Homo sapiens
SSNIGAGYY

SEQ ID NO: 39 - skipped

SEQ ID NO: 40 - protein, 11 aa, Homo sapiens
SAWDSSLSAVM

SEQ ID NO: 41 - protein, 120 aa, Homo sapiens
QLQLQESGPGVVKPSETLSLTCTISGGSFSTYYWTWIRQPPGKGLEWVGYIGNGGRSLNYNPSLKSRITLSVDASKNQFSLKVTSVTAADTAVYYCGRARGLRGNWFDVWGPGVLVTVSS

SEQ ID NO: 42 - DNA, 360 bp, Homo sapiens
  source 1..360: mol_type = genomic DNA
caactgcagttgcaggagtcgggcccaggagtggtgaagccttcggagaccctgtccctcacctgcactatctctggtggctccttcagtacttactactggacctggattcgccagcccccagggaagggactggagtgggttgggtatatcggtaatggtggtcgtagcctcaactacaacccctccctcaagagtcgcatcaccctgtcagtagacgcgtccaagaaccagttctccctgaaggtgacctctgtgaccgccgcggacacggccgtctattactgtgggagagccaggggactccgcggaaactggttcgatgtctggggcccgggagtcctggtcaccgtctcctca

SEQ ID NO: 43 - protein, 8 aa, Homo sapiens
GGSFSTYY

SEQ ID NO: 44 - protein, 8 aa, Homo sapiens
IGNGGRSL

SEQ ID NO: 45 - protein, 14 aa, Homo sapiens
GRARGLRGNWFDVW

SEQ ID NO: 46 - protein, 110 aa, Homo sapiens
QAALTQPPSVSGSPGQSVTISCTGTSSDIGGYNYVSWYQQHPGKAPKVMIYEVSKRPSGVSDRFSGSKSGNIASLTISGLQAEDEADYYCSSYAGSNTFLFGGGTRLTVL

SEQ ID NO: 47 - DNA, 330 bp, Homo sapiens
  source 1..330: mol_type = genomic DNA
caggctgccctgactcagcctccctctgtgtctgggtctcctggacagtcggtcaccatctcctgcactggaaccagcagtgacatcggtggttataactatgtctcctggtaccaacaacacccaggcaaagcccccaaagtcatgatttatgaggtcagtaagcggccctcaggggtctctgatcgcttctctggttccaaatctggcaacatagcctccctgaccatctctgggctccaggctgaggacgaggctgattattactgcagctcatatgcaggcagcaacactttcttattcggaggagggacccggctgacagtacta

SEQ ID NO: 48 - protein, 9 aa, Homo sapiens
SSDIGGYNY

SEQ ID NO: 49 - skipped

SEQ ID NO: 50 - protein, 10 aa, Homo sapiens
SSYAGSNTFL

SEQ ID NO: 51 - protein, 123 aa, Homo sapiens
QVQLQESGPGLVKPSETLSLTCAVSGGSISSNYWSWIRQPPGKGLEWIGRIYGSGGSTDYNPSLKSRVTISTDTSKNQFSLKVSSVTAADTAVYYCARVRIQWVQLRGWFDVWGPGVLVTVSS

SEQ ID NO: 52 - DNA, 369 bp, Homo sapiens
  source 1..369: mol_type = genomic DNA
caggtgcagctgcaggagtcgggcccaggactggtgaagccttcggagaccctgtccctcacctgcgctgtctctggtggctccatcagcagtaactactggagctggatccgccagcccccagggaagggactggagtggattggacgtatctatggtagtggtgggagcaccgactacaacccctccctcaagagtcgagtcaccatttcaacagacacgtccaagaaccagttctccctgaaggtgagctctgtgaccgccgcggacacggccgtgtattactgtgcgagagtgcggatacagtgggtacagttgcgaggctggttcgatgtctggggcccgggagtcctggtcaccgtctcctca

SEQ ID NO: 53 - protein, 10 aa, Homo sapiens
GGSISSNYWS

SEQ ID NO: 54 - protein, 8 aa, Homo sapiens
IYGSGGST

SEQ ID NO: 55 - protein, 17 aa, Homo sapiens
ARVRIQWVQLRGWFDVW

SEQ ID NO: 56 - protein, 107 aa, Homo sapiens
YIQMTQSPSSLSASVGDTVTFTGPASQSFSSSLAWYQQKPGKAPNLLIYSASSLQCGVRSRFSGSKSGTDFTLTISSLQPEDIASYYCQQYYSYPFTFGPGTKLDIK

SEQ ID NO: 57 - DNA, 321 bp, Homo sapiens
  source 1..321: mol_type = genomic DNA
tacatacagatgacgcagtctccatcctccctgtctgcatctgtaggagacacagtcaccttcactggccccgcaagtcagagctttagtagtagtttagcctggtatcagcagaaaccagggaaagcccctaacctcctgatctatagtgcatccagtttgcaatgtggggttcgttcgaggttcagtggcagtaagtctgggacagatttcactctcaccatcagcagcctgcagcctgaagatattgctagttattactgtcaacagtattacagttatccattcactttcggccccgggaccaaactggatatcaaa

SEQ ID NO: 58 - protein, 6 aa, Homo sapiens
QSFSSS

SEQ ID NO: 59 - skipped

SEQ ID NO: 60 - protein, 9 aa, Homo sapiens
QQYYSYPFT

SEQ ID NO: 61 - protein, 119 aa, Homo sapiens
QVQLQESGPGLVRPSETLSLTCAVSGGSISSNYWSWIRQPPGKGLEWIGYISGSTGSTYQNPSLKSRVTVSKDTSKNQFSLKLNSVTAADTAVYYCARSGRRGSSLDLWGRGVLVTVSS

SEQ ID NO: 62 - DNA, 357 bp, Homo sapiens
  source 1..357: mol_type = genomic DNA
caggtgcagctgcaggagtcgggcccaggactggtgaggccttcggagaccctatccctcacctgcgctgtctctggtggctccatcagcagtaactactggagctggattcgccagcccccagggaaggggctggagtggattgggtatatctctggtagtactgggagcacctaccagaacccctccctcaagagtcgagtcaccgtttcaaaagacacgtctaagaaccagttctccctgaagctgaattctgtgaccgccgcggacacggccgtgtattactgtgcgagaagtgggagaagaggcagctcattggatttgtggggccggggagttctggtcaccgtctcctca

SEQ ID NO: 63 - protein, 8 aa, Homo sapiens
GGSISSNY

SEQ ID NO: 64 - protein, 8 aa, Homo sapiens
ISGSTGST

SEQ ID NO: 65 - protein, 13 aa, Homo sapiens
ARSGRRGSSLDLW

SEQ ID NO: 66 - protein, 111 aa, Homo sapiens
QSVLTQPPSVSGDPGQRVTISCTGSSSNIGAGYYVYWYQQFPGTAPKLLIYQDNKRPSGVSDRFSGSKSGTSASLTITGLQPGDEADYYCSAWDSSLSAVFFGGGTRLTVL

SEQ ID NO: 67 - DNA, 333 bp, Homo sapiens
  source 1..333: mol_type = genomic DNA
cagtctgtgctgacgcagccgccctcagtgtctggggaccccgggcagagggtcaccatctcgtgcactgggagcagctccaacatcggggcgggttattatgtatactggtaccagcagttcccaggaacggcccccaaactcctcatctatcaagataataagcgaccctcaggggtttctgaccgattctctggctccaagtctggtacctcagcctccctgaccatcactgggctccagcctggggatgaggctgattattactgctcagcatgggatagcagcctgagtgctgtgttcttcggaggagggacccggctgacagtacta

SEQ ID NO: 68 - protein, 9 aa, Homo sapiens
SSNIGAGYY

SEQ ID NO: 69 - skipped

SEQ ID NO: 70 - protein, 11 aa, Homo sapiens
SAWDSSLSAVF

SEQ ID NO: 71 - protein, 121 aa, Homo sapiens
QLQESGPGLVKPSETLSLTCTVSGGSISDTYRWSWIRQSPGKGLEWIAYIYGTTTSTNYNPSLKSRLTISKDTSKNQFSLNLRSVTAADTAVYYCARGDSGGRSAHVFHFWGQGLRVTVSS

SEQ ID NO: 72 - DNA, 363 bp, Homo sapiens
  source 1..363: mol_type = genomic DNA
cagctgcaggagtcgggcccaggactggtgaagccttcggagaccctgtccctcacctgcactgtctctggtggctccatcagcgatacttaccggtggagctggattcgccagtccccagggaagggactggagtggattgcctacatctatggtactactacgagcaccaactacaacccctccctcaagagtcgactcaccatttcaaaagacacgtccaagaaccagttctccttgaacctgaggtctgtgaccgccgcggacacggccgtgtattactgtgcgagaggggatagcggtggccggtcagcgcatgtttttcatttctggggccaagggctcagggtcaccgtctcttca

SEQ ID NO: 73 - protein, 9 aa, Homo sapiens
GGSISDTYR

SEQ ID NO: 74 - protein, 8 aa, Homo sapiens
IYGTTTST

SEQ ID NO: 75 - protein, 16 aa, Homo sapiens
ARGDSGGRSAHVFHFW

SEQ ID NO: 76 - protein, 111 aa, Homo sapiens
QSVLTQPPSVFGDPGQRITISCTGSSSNIGAGYYVYWYQQFPGTAPKLLIYQDNKRPSGVSDRFSGSKSGSSASLTITGLQPGDEADYYCSAWDSSLSVRVFGGGTRLTVL

SEQ ID NO: 77 - DNA, 333 bp, Homo sapiens
  source 1..333: mol_type = genomic DNA
cagagtgttctgacgcagccgccctcagtgtttggggaccccgggcagaggatcaccatctcgtgcactgggagcagctccaacatcggggcgggttattatgtatactggtaccagcagttcccaggaacggcccccaaactcctcatctatcaagataataagcgaccctcaggggtttctgaccgattttctggctccaagtctggttcctcagcctccctgaccatcactgggctccagcctggggatgaggctgattattactgctcagcatgggatagcagcctgagtgtacgggttttcggaggagggacccggctgacagtacta

SEQ ID NO: 78 - protein, 9 aa, Homo sapiens
SSNIGAGYY

SEQ ID NO: 79 - skipped

SEQ ID NO: 80 - protein, 11 aa, Homo sapiens
SAWDSSLSVRV

SEQ ID NO: 81 - protein, 122 aa, Homo sapiens
EVQLVESGGGLVQPGGSLRLSCAASGFTFSSYGMNWVRQAPGKGLEWVSFITNTGKTTYYADSVRGRFTISRDNAKKSVSLQMSSLRAEDTAVYYCTRGRGRHGWSSGVFDFWGQGLRVTVS

SEQ ID NO: 82 - DNA, 368 bp, Homo sapiens
  source 1..368: mol_type = genomic DNA
gaggtgcaactggtggagtctggaggaggcttggtccagcctggagggtccctgagactctcctgtgcagcctctggattcaccttcagtagttacggcatgaactgggtccgccaggctccgggaaaggggctggagtgggtctcattcattactaacactggtaaaaccacatactacgctgactctgtgaggggccgattcaccatctccagagacaacgccaagaagtcggtgtctctacaaatgagtagcctgagagccgaggacacggccgtctattactgtactaggggaagaggtagacacggctggtccagtggtgtttttgatttctggggccaaggtctcagggtcaccgtctcttc

SEQ ID NO: 83 - protein, 8 aa, Homo sapiens
GFTFSSYG

SEQ ID NO: 84 - protein, 8 aa, Homo sapiens
ITNTGKTT

SEQ ID NO: 85 - protein, 16 aa, Homo sapiens
TGRGRHGWSSGVFDFW

SEQ ID NO: 86 - protein, 111 aa, Homo sapiens
QSVLTQPPSVFGDPGQRITISCTGSSSNIGAGYYVYWYQQFPGTAPKLLIYQDNKRPSGVSDRFSGSKFGSSASLTITGVQRGDEGDYYCSAWDSSLSVRVLGGGTRLTVL

SEQ ID NO: 87 - DNA, 333 bp, Homo sapiens
  source 1..333: mol_type = genomic DNA
cagtctgttctgacgcagccgccctcagtgttcggggaccccgggcagaggatcaccatttcgtgcactgggagcagctccaacatcggggcgggttattatgtatactggtaccagcagttcccaggaacggcccccaaactcctcatctatcaagataataagcgaccctcaggggtttctgaccgattctctggctccaagtttggttcctcagcctccctgaccatcactggggtccagcgtggggatgagggtgattattactgctcagcatgggatagcagcctgagtgtacgggttttgggaggagggacccggctgacagtacta

SEQ ID NO: 88 - protein, 9 aa, Homo sapiens
SSNIGAGYY

SEQ ID NO: 89 - skipped

SEQ ID NO: 90 - protein, 11 aa, Homo sapiens
SAWDSSLSVRV

SEQ ID NO: 91 - protein, 121 aa, Homo sapiens
EVQLVESGGGLVQPGGSLRLSCVASGFTFSDRYIDWVRQAPGKGLEWVSTISTGSGDTALYSDSVKGRFTISRDNAKNTLYLQMNSLRAEDTAVYYCARHSGTFYTHFDYWGQGVLVTVSS

SEQ ID NO: 92 - DNA, 363 bp, Homo sapiens
  source 1..363: mol_type = genomic DNA
gaagtgcagttggtggagtctgggggaggcttggtacagccgggggggtccctgagactctcctgtgtagcctctggattcaccttcagtgaccgctacatagactgggtccgccaggctccagggaagggcctggagtgggtctcaactattagcactggtagtggtgataccgcattgtactcagactctgtcaagggccgattcaccatctccagagacaacgccaagaacacactgtatctgcaaatgaacagcctgagagccgaagacacggctgtctattactgtgcgagacatagtggtactttttacacccactttgactactggggccagggagtcctggtcaccgtctcctca

SEQ ID NO: 93 - protein, 8 aa, Homo sapiens
GFTFSDRY

SEQ ID NO: 94 - protein, 9 aa, Homo sapiens
ISTGSGDTA

SEQ ID NO: 95 - protein, 14 aa, Homo sapiens
ARHSGTFYTHFDYW

SEQ ID NO: 96 - protein, 107 aa, Homo sapiens
DIQMTQSPSSLSASVGDTVTFTCRASRSISSWLAWYQQKPGRAPKVLIYKASSLQSGVPSRFSGSGSGTDFTLTISSLQSEDFATYYCQQYSSRPPTFGQGTKVEIR

SEQ ID NO: 97 - DNA, 321 bp, Homo sapiens
  source 1..321: mol_type = genomic DNA
gacatccagatgacccagtctccatcctccctgtctgcatctgtaggagacacagtcaccttcacctgccgggcgagtcggagtattagcagctggttagcctggtatcagcagaaaccagggagagcccctaaagtcctgatctataaggcgtccagtttgcaaagtggggttccttcaaggttcagcggcagtggatctgggacagacttcactctcaccatcagcagcctacagtctgaagattttgcaacatattattgtcaacagtatagtagtcgccctccgacgttcggccaagggaccaaggtggaaatcaga

SEQ ID NO: 98 - protein, 6 aa, Homo sapiens
RSISSW

SEQ ID NO: 99 - skipped

SEQ ID NO: 100 - protein, 9 aa, Homo sapiens
QQYSSRPPT

SEQ ID NO: 101 - protein, 119 aa, Homo sapiens
QVQLQESGPGLLKPSETLSLTCAVSGGSFSSFWWSWLRQPPEKGLEWIGEINGDSGSTNYNPSLKSRVTISKDASKNQFSLKLTSVTAADTAVFYCARVRRILRSLDVWGRGVLVTVSS

SEQ ID NO: 102 - DNA, 357 bp, Homo sapiens
  source 1..357: mol_type = genomic DNA
caggtgcagctgcaggagtcgggcccaggactgctgaagccttcggagaccctgtccctcacctgcgctgtctctggtggctccttcagtagtttctggtggagctggctccgccagcccccagaaaagggactggagtggattggggagatcaatggtgatagtgggagcaccaactacaacccctccctcaagagtcgagtcaccatttcaaaagacgcgtccaagaaccagttctccctgaaactgacctctgtgaccgccgcggacacggccgttttttactgtgcgagagttcggcgaattctgaggtcattggatgtctggggccggggagttctggtcaccgtctcctca

SEQ ID NO: 103 - protein, 8 aa, Homo sapiens
GGSFSSFW

SEQ ID NO: 104 - protein, 8 aa, Homo sapiens
INGDSGST

SEQ ID NO: 105 - protein, 13 aa, Homo sapiens
ARVRRILRSLDVW

SEQ ID NO: 106 - protein, 107 aa, Homo sapiens
DIQMTQSPFSLFAFVGDRVTITCQASQGISHLLAWYQQKPGKAPKLLIYSASTLQSGVPSRFSGSGFGTEFTLTISSLQPEDFATYYCQQHNSYPRTFGQGTKVEIK

SEQ ID NO: 107 - DNA, 321 bp, Homo sapiens
  source 1..321: mol_type = genomic DNA
gacatccagatgacccagtctcctttttccttgtttgcatttgtaggagacagagtcaccatcacttgccaagccagtcagggtattagccacttgttagcttggtatcagcagaaaccagggaaagcccctaagctccttatttattctgcatccactttgcaaagtggggtcccatcaaggttcagcggcagtggatttgggacggaattcactctcaccatcagcagcctgcagcctgaagattttgcaacttattactgtcaacagcataatagttaccctcggacgttcggccaagggaccaaggtggaaatcaaa

SEQ ID NO: 108 - protein, 6 aa, Homo sapiens
QGISHL

SEQ ID NO: 109 - skipped

SEQ ID NO: 110 - protein, 9 aa, Homo sapiens
QQHNSYPRT

SEQ ID NO: 111 - DNA, 5845 bp, Homo sapiens
  source 1..5845: mol_type = genomic DNA
tcgcgcgtttcggtgatgacggtgaaaacctctgacacatgcagctcccggagacggtcacagcttgtctgtaagcggatgccgggagcagacaagcccgtcagggcgcgtcagcgggtgttggcgggtgtcggggctggcttaactatgcggcatcagagcagattgtactgagagtgcaccatatgcggtgtgaaataccgcacagatgcgtaaggagaaaataccgcatcagattggctattggccattgcatacgttgtatccatatcataatatgtacatttatattggctcatgtccaacattaccgccatgttgacattgattattgactagttattaatagtaatcaattacggggtcattagttcatagcccatatatggagttccgcgttacataacttacggtaaatggcccgcctggctgaccgcccaacgacccccgcccattgacgtcaataatgacgtatgttcccatagtaacgccaatagggactttccattgacgtcaatgggtggagtatttacggtaaactgcccacttggcagtacatcaagtgtatcatatgccaagtacgccccctattgacgtcaatgacggtaaatggcccgcctggcattatgcccagtacatgaccttatgggactttcctacttggcagtacatctacgtattagtcatcgctattaccatggtgatgcggttttggcagtacatcaatgggcgtggatagcggtttgactcacggggatttccaagtctccaccccattgacgtcaatgggagtttgttttggcaccaaaatcaacgggactttccaaaatgtcgtaacaactccgccccattgacgcaaatgggcggtaggcgtgtacggtgggaggtctatataagcagagctcgtttagtgaaccgtcagatcgcctggagacgccatccacgctgttttgacctccatagaagacaccgggaccgatccagcctccatcggctcgcatctctccttcacgcgcccgccgccctacctgaggccgccatccacgccggttgagtcgcgttctgccgcctcccgcctgtggtgcctcctgaactgcgtccgccgtctaggtaagtttaaagctcaggtcgagaccgggcctttgtccggcgctcccttggagcctacctagactcagccggctctccacgctttgcctgaccctgcttgctcaactctagttaacggtggagggcagtgtagtctgagcagtactcgttgctgccgcgcgcgccaccagacataatagctgacagactaacagactgttcctttccatgggtcttttctgcagtcaccgtcgtcgacacgtgtgatcagatatcgcggccgctctagaccaccatgggatggtcatgtatcatcctttttctagtagcaactgcaaccggtgtacattcccaggtgcagctggtgcagctgcacgagtcgggcccaggactggtgaagccttcggagaccctgtccctcacctgcgctgtctctggtggctctatcagcagtagctactggagctggatccgccaggccccagggaagggactggagtggattgggtatgtctatggtagtggtcgtgacaccaacgacaacccctccctcaagagtcgagtcaccctgtcagtagacacgtccaagaaccagctctccctgaagctgagatctgtgaccgccgcggacacggccgtgtattactgtgcgagcagcggctggcctcctgggttggactactggggccagggagtcacggtcaccgtctcctcagctagcaccaagggccctagtgtgtttcctctggcccctagcagcagaagcacatctgaatctacagccgccctgggctgcctggtgaaagattacttccccgagcccgtgaccgtgtcttggaatagcggctctctgaccagcggcgtgcacacatttccagctgtgctgcagagcagcggcctgtattctctgagcagcgtggtgacagtgccaagcagctctctgggcacccagacctacgtgtgcaacgtgaaccacaagcccagcaacaccaaggtggacaagcgggtggaaatcaagacctgtggcggcggaagcaagcctcctacctgtcctccttgtaccagccctgaactgctgggcggacctagcgtgttcctgttccccccaaagcccaaggacaccctgatgatcagcagaacccccgaagtgacctgcgtggtggtggatgtgtcccaggaagatcccgacgtgaagttcaattggtacgtgaacggcgccgaggtgcaccatgcccagacaaagcccagagagacacagtacaacagcacctaccgggtggtgtctgtgctgaccgtgacacaccaggactggctgaacggcaaagagtacacatgcaaggtgtccaacaaggccctgcctgcccccatccagaaaaccatcagcaaggacaagggccagcccagagaacctcaggtgtacacactgccccccagcagagaggaactgaccaagaatcaggtgtccctgacctgtctggtgaaaggcttctaccccagcgacatcgtggtggaatgggagtctagcggacagcccgagaacacctacaagaccacccctccagtgctggatagcgacggcagctacttcctgtacagcaagctgaccgtggacaagagcagatggcagcagggcaacgtgttcagctgctctgtgatgcacgaggccctgcacaaccactacacccagaagtctctgagcctgagccccggaaagtgatgatgaacacgtgggatccagatctgctgtgccttctagttgccagccatctgttgtttgcccctcccccgtgccttccttgaccctggaaggtgccactcccactgtcctttcctaataaaatgaggaaattgcatcgcattgtctgagtaggtgtcattctattctggggggtggggtggggcaggacagcaagggggaggattgggaagacaatagcaggcatgctggggatgcggtgggctctatgggtacccaggtgctgaagaattgacccggttcctcctgggccagaaagaagcaggcacatccccttctctgtgacacaccctgtccacgcccctggttcttagttccagccccactcataggacactcatagctcaggagggctccgccttcaatcccacccgctaaagtacttggagcggtctctccctccctcatcagcccaccaaaccaaacctagcctccaagagtgggaagaaattaaagcaagataggctattaagtgcagagggagagaaaatgcctccaacatgtgaggaagtaatgagagaaatcatagaattttaaggccatgatttaaggccatcatggccttaatcttccgcttcctcgctcactgactcgctgcgctcggtcgttcggctgcggcgagcggtatcagctcactcaaaggcggtaatacggttatccacagaatcaggggataacgcaggaaagaacatgtgagcaaaaggccagcaaaaggccaggaaccgtaaaaaggccgcgttgctggcgtttttccataggctccgcccccctgacgagcatcacaaaaatcgacgctcaagtcagaggtggcgaaacccgacaggactataaagataccaggcgtttccccctggaagctccctcgtgcgctctcctgttccgaccctgccgcttaccggatacctgtccgcctttctcccttcgggaagcgtggcgctttctcatagctcacgctgtaggtatctcagttcggtgtaggtcgttcgctccaagctgggctgtgtgcacgaaccccccgttcagcccgaccgctgcgccttatccggtaactatcgtcttgagtccaacccggtaagacacgacttatcgccactggcagcagccactggtaacaggattagcagagcgaggtatgtaggcggtgctacagagttcttgaagtggtggcctaactacggctacactagaagaacagtatttggtatctgcgctctgctgaagccagttaccttcggaaaaagagttggtagctcttgatccggcaaacaaaccaccgctggtagcggtggtttttttgtttgcaagcagcagattacgcgcagaaaaaaaggatctcaagaagatcctttgatcttttctacggggtctgacgctcagtggaacgaaaactcacgttaagggattttggtcatgagattatcaaaaaggatcttcacctagatccttttaaattaaaaatgaagttttaaatcaatctaaagtatatatgagtaaacttggtctgacagttaccaatgcttaatcagtgaggcacctatctcagcgatctgtctatttcgttcatccatagttgcctgactcggggggggggggcgctgaggtctgcctcgtgaagaaggtgttgctgactcataccaggcctgaatcgccccatcatccagccagaaagtgagggagccacggttgatgagagctttgttgtaggtggaccagttggtgattttgaacttttgctttgccacggaacggtctgcgttgtcgggaagatgcgtgatctgatccttcaactcagcaaaagttcgatttattcaacaaagccgccgtcccgtcaagtcagcgtaatgctctgccagtgttacaaccaattaaccaattctgattagaaaaactcatcgagcatcaaatgaaactgcaatttattcatatcaggattatcaataccatatttttgaaaaagccgtttctgtaatgaaggagaaaactcaccgaggcagttccataggatggcaagatcctggtatcggtctgcgattccgactcgtccaacatcaatacaacctattaatttcccctcgtcaaaaataaggttatcaagtgagaaatcaccatgagtgacgactgaatccggtgagaatggcaaaagcttatgcatttctttccagacttgttcaacaggccagccattacgctcgtcatcaaaatcactcgcatcaaccaaaccgttattcattcgtgattgcgcctgagcgagacgaaatacgcgatcgctgttaaaaggacaattacaaacaggaatcgaatgcaaccggcgcaggaacactgccagcgcatcaacaatattttcacctgaatcaggatattcttctaatacctggaatgctgttttcccggggatcgcagtggtgagtaaccatgcatcatcaggagtacggataaaatgcttgatggtcggaagaggcataaattccgtcagccagtttagtctgaccatctcatctgtaacatcattggcaacgctacctttgccatgtttcagaaacaactctggcgcatcgggcttcccatacaatcgatagattgtcgcacctgattgcccgacattatcgcgagcccatttatacccatataaatcagcatccatgttggaatttaatcgcggcctcgagcaagacgtttcccgttgaatatggctcataacaccccttgtattactgtttatgtaagcagacagttttattgttcatgatgatatatttttatcttgtgcaatgtaacatcagagattttgagacacaacgtggctttccccccccccccattattgaagcatttatcagggttattgtctcatgagcggatacatatttgaatgtatttagaaaaataaacaaataggggttccgcgcacatttccccgaaaagtgccacctgacgtctaagaaaccattattatcatgacattaacctataaaaataggcgtatcacgaggccctttcgtc

SEQ ID NO: 112 - protein, 473 aa, Homo sapiens
MGWSCIILFLVATATGVHSQVQLVQLHESGPGLVKPSETLSLTCAVSGGSISSSYWSWIRQAPGKGLEWIGYVYGSGRDTNDNPSLKSRVTLSVDTSKNQLSLKLRSVTAADTAVYYCASSGWPPGLDYWGQGVTVTVSSASTKGPSVFPLAPSSRSTSESTAALGCLVKDYFPEPVTVSWNSGSLTSGVHTFPAVLQSSGLYSLSSVVTVPSSSLGTQTYVCNVNHKPSNTKVDKRVEIKTCGGGSKPPTCPPCTSPELLGGPSVFLFPPKPKDTLMISRTPEVTCVVVDVSQEDPDVKFNWYVNGAEVHHAQTKPRETQYNSTYRVVSVLTVTHQDWLNGKEYTCKVSNKALPAPIQKTISKDKGQPREPQVYTLPPSREELTKNQVSLTCLVKGFYPSDIVVEWESSGQPENTYKTTPPVLDSDGSYFLYSKLTVDKSRWQQGNVFSCSVMHEALHNHYTQKSLSLSPGK

SEQ ID NO: 113 - DNA, 5100 bp, Homo sapiens
  source 1..5100: mol_type = genomic DNA
tcgcgcgtttcggtgatgacggtgaaaacctctgacacatgcagctcccggagacggtcacagcttgtctgtaagcggatgccgggagcagacaagcccgtcagggcgcgtcagcgggtgttggcgggtgtcggggctggcttaactatgcggcatcagagcagattgtactgagagtgcaccatatgcggtgtgaaataccgcacagatgcgtaaggagaaaataccgcatcagattggctattggccattgcatacgttgtatccatatcataatatgtacatttatattggctcatgtccaacattaccgccatgttgacattgattattgactagttattaatagtaatcaattacggggtcattagttcatagcccatatatggagttccgcgttacataacttacggtaaatggcccgcctggctgaccgcccaacgacccccgcccattgacgtcaataatgacgtatgttcccatagtaacgccaatagggactttccattgacgtcaatgggtggagtatttacggtaaactgcccacttggcagtacatcaagtgtatcatatgccaagtacgccccctattgacgtcaatgacggtaaatggcccgcctggcattatgcccagtacatgaccttatgggactttcctacttggcagtacatctacgtattagtcatcgctattaccatggtgatgcggttttggcagtacatcaatgggcgtggatagcggtttgactcacggggatttccaagtctccaccccattgacgtcaatgggagtttgttttggcaccaaaatcaacgggactttccaaaatgtcgtaacaactccgccccattgacgcaaatgggcggtaggcgtgtacggtgggaggtctatataagcagagctcgtttagtgaaccgtcagatcgcctggagacgccatccacgctgttttgacctccatagaagacaccgggaccgatccagcctccatcggctcgcatctctccttcacgcgcccgccgccctacctgaggccgccatccacgccggttgagtcgcgttctgccgcctcccgcctgtggtgcctcctgaactgcgtccgccgtctaggtaagtttaaagctcaggtcgagaccgggcctttgtccggcgctcccttggagcctacctagactcagccggctctccacgctttgcctgaccctgcttgctcaactctagttaacggtggagggcagtgtagtctgagcagtacacgttgctgccgcgcgcgccaccagacataatagctgacagactaacagactgttcctttccatgggtcttttctgcagtcaccgtcgtcgacacgtgtgatcagatatcgcggccgctctagaccaccatgggatggtcatgtatcatcctttttctagtagcaactgcaaccggtgtacattcagaaattgtgttgacacagtctccaggcaccctgtctttgtctccaggggaaacagccatcatctcttgtcggaccagtcagtatggttccttagcctggtatcaacagaggcccggccaggcccccaggctcgtcatctattcgggctctactcgggccgctggcatcccagacaggttcagcggcagtcggtgggggccagactacaatctcaccatcagcaacctggagtcgggagattttggtgtttattattgccagcagtatgaattttttggccaggggaccaaggtccaggtcgacattaaacgtacggtggctgcaccatctgtcttcatcttcccgccatctgaggatcaggtgaaatctggaactgtctctgttgtgtgcctgctgaataacttctatcccagagaggccagcgtaaagtggaaggtggatggtgccctcaaaacgggtaactcccaggagagtgtcacagagcaggacagcaaggacaacacctacagcctgagcagcaccctgacgctgagcagcacagagtaccagagtcacaaagtctatgcctgcgaagtcacccatcagggcctgagctcgcccgtcaccaagagcttcaacagaggagagtgttagggatccagatctgctgtgccttctagttgccagccatctgttgtttgcccctcccccgtgccttccttgaccctggaaggtgccactcccactgtcctttcctaataaaatgaggaaattgcatcgcattgtctgagtaggtgtcattctattctggggggtggggtggggcaggacagcaagggggaggattgggaagacaatagcaggcatgctggggatgcggtgggctctatgggtacccaggtgctgaagaattgacccggttcctcctgggccagaaagaagcaggcacatccccttctctgtgacacaccctgtccacgcccctggttcttagttccagccccactcataggacactcatagctcaggagggctccgccttcaatcccacccgctaaagtacatggagcggtctctccctccctcatcagcccaccaaaccaaacctagcctccaagagtgggaagaaattaaagcaagataggctattaagtgcagagggagagaaaatgcctccaacatgtgaggaagtaatgagagaaatcatagaattttaaggccatgatttaaggccatcatggccttaatcttccgcttcctcgctcactgactcgctgcgctcggtcgttcggctgcggcgagcggtatcagctcactcaaaggcggtaatacggttatccacagaatcaggggataacgcaggaaagaacatgtgagcaaaaggccagcaaaaggccaggaaccgtaaaaaggccgcgttgctggcgtttttccataggctccgcccccctgacgagcatcacaaaaatcgacgctcaagtcagaggtggcgaaacccgacaggactataaagataccaggcgtttccccctggaagctccctcgtgcgctctcctgttccgaccctgccgcttaccggatacctgtccgcctttctcccttcgggaagcgtggcgctttctcatagctcacgctgtaggtatctcagttcggtgtaggtcgttcgctccaagctgggctgtgtgcacgaaccccccgttcagcccgaccgctgcgccttatccggtaactatcgtcttgagtccaacccggtaagacacgacttatcgccactggcagcagccactggtaacaggattagcagagcgaggtatgtaggcggtgctacagagttcttgaagtggtggcctaactacggctacactagaagaacagtatttggtatctgcgctctgctgaagccagttaccttcggaaaaagagttggtagctcttgatccggcaaacaaaccaccgctggtagcggtggtttttttgtttgcaagcagcagattacgcgcagaaaaaaaggatctcaagaagatcctttgatcttttctacggggtctgacgctcagtggaacgaaaactcacgttaagggattttggtcatgagattatcaaaaaggatcttcacctagatccttttaaattaaaaatgaagttttaaatcaatctaaagtatatatgagtaaacttggtctgacagttaccaatgcttaatcagtgaggcacctatctcagcgatctgtctatttcgttcatccatagttgcctgactcggggggggggggcgctgaggtctgcctcgtgaagaaggtgttgctgactcataccaggcctgaatcgccccatcatccagccagaaagtgagggagccacggttgatgagagctttgttgtaggtggaccagttggtgattttgaacttttgctttgccacggaacggtctgcgttgtcgggaagatgcgtgatctgatccttcaactcagcaaaagttcgatttattcaacaaagccgccgtcccgtcaagtcagcgtaatgctctgccagtgttacaaccaattaaccaattctgattagaaaaactcatcgagcatcaaatgaaactgcaatttattcatatcaggattatcaataccatatttttgaaaaagccgtttctgtaatgaaggagaaaactcaccgaggcagttccataggatggcaagatcctggtatcggtctgcgattccgactcgtccaacatcaatacaacctattaatttcccctcgtcaaaaataaggttatcaagtgagaaatcaccatgagtgacgactgaatccggtgagaatggcaaaagcttatgcatttctttccagacttgttcaacaggccagccattacgctcgtcatcaaaatcactcgcatcaaccaaaccgttattcattcgtgattgcgcctgagcgagacgaaatacgcgatcgctgttaaaaggacaattacaaacaggaatcgaatgcaaccggcgcaggaacactgccagcgcatcaacaatattttcacctgaatcaggatattcttctaatacctggaatgctgttttcccggggatcgcagtggtgagtaaccatgcatcatcaggagtacggataaaatgcttgatggtcggaagaggcataaattccgtcagccagtttagtctgaccatctcatctgtaacatcattggcaacgctacctttgccatgtttcagaaacaactctggcgcatcgggcttcccatacaatcgatagattgtcgcacctgattgcccgacattatcgcgagcccatttatacccatataaatcagcatccatgttggaatttaatcgcggcctcgagcaagacgtttcccgttgaatatggctcataacaccccttgtattactgtttatgtaagcagacagttttattgttcatgatgatatatttttatcttgtgcaatgtaacatcagagattttgagacacaacgtggctttccccccccccccattattgaagcatttatcagggttattgtctcatgagcggatacatatttgaatgtatttagaaaaataaacaaataggggttccgcgcacatttccccgaaaagtgccacctgacgtctaagaaaccattattatcatgacattaacctataaaaataggcgtatcacgaggccctttcgtc

SEQ ID NO: 114 - protein, 229 aa, Homo sapiens
MGWSCIILFLVATATGVHSEIVLTQSPGTLSLSPGETAIISCRTSQYGSLAWYQQRPGQAPRLVIYSGSTRAAGIPDRFSGSRWGPDYNLTISNLESGDFGVYYCQQYEFFGQGTKVQVDIKRTVAAPSVFIFPPSEDQVKSGTVSVVCLLNNFYPREASVKWKVDGALKTGNSQESVTEQDSKDNTYSLSSTLTLSSTEYQSHKVYACEVTHQGLSSPVTKSFNRGEC

SEQ ID NO: 115 - protein, 235 aa, Homo sapiens
MGWSCIILFLVATATGVHSQSALTQPPSVSGSPGQSVTISCTGTSSDVDGYNYVSWYQQHPGKAPKLMIYGVSNRPSGVSDRFSGSKSGNTASLTISGLQAEDEADYYCCSSTTSYTYIFGTGTKVTVLGQPKAAPSVTLFPPSSEELQANKATLVCLISDFYPGAVEVAWKADGSAVNAGVETTKPSKQSNNKYAASSYLSLTSDQWKSHKSYSCQVTHEGSTVEKTVAPAECS

SEQ ID NO: 116 - DNA, 5842 bp, Homo sapiens
  source 1..5842: mol_type = genomic DNA
tcgcgcgtttcggtgatgacggtgaaaacctctgacacatgcagctcccggagacggtcacagcttgtctgtaagcggatgccgggagcagacaagcccgtcagggcgcgtcagcgggtgttggcgggtgtcggggctggcttaactatgcggcatcagagcagattgtactgagagtgcaccatatgcggtgtgaaataccgcacagatgcgtaaggagaaaataccgcatcagattggctattggccattgcatacgttgtatccatatcataatatgtacatttatattggctcatgtccaacattaccgccatgttgacattgattattgactagttattaatagtaatcaattacggggtcattagttcatagcccatatatggagttccgcgttacataacttacggtaaatggcccgcctggctgaccgcccaacgacccccgcccattgacgtcaataatgacgtatgttcccatagtaacgccaatagggactttccattgacgtcaatgggtggagtatttacggtaaactgcccacttggcagtacatcaagtgtatcatatgccaagtacgccccctattgacgtcaatgacggtaaatggcccgcctggcattatgcccagtacatgaccttatgggactttcctacttggcagtacatctacgtattagtcatcgctattaccatggtgatgcggttttggcagtacatcaatgggcgtggatagcggtttgactcacggggatttccaagtctccaccccattgacgtcaatgggagtttgttttggcaccaaaatcaacgggactttccaaaatgtcgtaacaactccgccccattgacgcaaatgggcggtaggcgtgtacggtgggaggtctatataagcagagctcgtttagtgaaccgtcagatcgcctggagacgccatccacgctgttttgacctccatagaagacaccgggaccgatccagcctccatcggctcgcatctctccttcacgcgcccgccgccctacctgaggccgccatccacgccggttgagtcgcgttctgccgcctcccgcctgtggtgcctcctgaactgcgtccgccgtctaggtaagtttaaagctcaggtcgagaccgggcctttgtccggcgctcccttggagcctacctagactcagccggctctccacgctttgcctgaccctgcttgctcaactctagttaacggtggagggcagtgtagtctgagcagtactcgttgctgccgcgcgcgccaccagacataatagctgacagactaacagactgttcctttccatgggtcttttctgcagtcaccgtcgtcgacacgtgtgatcagatatcgcggccgctctagaccaccatgggatggtcatgtatcatcctttttctagtagcaactgcaaccggtgtacattcccaactgcagttgcaggagtcgggcccaggagtggtgaagccttcggagaccctgtccctcacctgcactatctctggtggctccttcagtacttactactggacctggattcgccagcccccagggaagggactggagtgggttgggtatatcggtaatggtggtcgtagcctcaactacaacccctccctcaagagtcgcatcaccctgtcagtagacgcgtccaagaaccagttctccctgaaggtgacctctgtgaccgccgcggacacggccgtctattactgtgggagagccaggggactccgcggaaactggttcgatgtctggggcccgggagtcctggtcaccgtctcctcagctagcaccaagggccctagtgtgtttcctctggcccctagcagcagaagcacatctgaatctacagccgccctgggctgcctggtgaaagattacttccccgagcccgtgaccgtgtcttggaatagcggctctctgaccagcggcgtgcacacatttccagctgtgctgcagagcagcggcctgtattctctgagcagcgtggtgacagtgccaagcagctctctgggcacccagacctacgtgtgcaacgtgaaccacaagcccagcaacaccaaggtggacaagcgggtggaaatcaagacctgtggcggcggaagcaagcctcctacctgtcctccttgtaccagccctgaactgctgggcggacctagcgtgttcctgttccccccaaagcccaaggacaccctgatgatcagcagaacccccgaagtgacctgcgtggtggtggatgtgtcccaggaagatcccgacgtgaagttcaattggtacgtgaacggcgccgaggtgcaccatgcccagacaaagcccagagagacacagtacaacagcacctaccgggtggtgtctgtgctgaccgtgacacaccaggactggctgaacggcaaagagtacacatgcaaggtgtccaacaaggccctgcctgcccccatccagaaaaccatcagcaaggacaagggccagcccagagaacctcaggtgtacacactgccccccagcagagaggaactgaccaagaatcaggtgtccctgacctgtctggtgaaaggcttctaccccagcgacatcgtggtggaatgggagtctagcggacagcccgagaacacctacaagaccacccctccagtgctggatagcgacggcagctacttcctgtacagcaagctgaccgtggacaagagcagatggcagcagggcaacgtgttcagctgctctgtgatgcacgaggccctgcacaaccactacacccagaagtctctgagcctgagccccggaaagtgatgatgaacacgtgggatccagatctgctgtgccttctagttgccagccatctgttgtttgcccctcccccgtgccttccttgaccctggaaggtgccactcccactgtcctttcctaataaaatgaggaaattgcatcgcattgtctgagtaggtgtcattctattctggggggtggggtggggcaggacagcaagggggaggattgggaagacaatagcaggcatgctggggatgcggtgggctctatgggtacccaggtgctgaagaattgacccggttcctcctgggccagaaagaagcaggcacatccccttctctgtgacacaccctgtccacgcccctggttcttagttccagccccactcataggacactcatagctcaggagggctccgccttcaatcccacccgctaaagtacttggagcggtctctccctccctcatcagcccaccaaaccaaacctagcctccaagagtgggaagaaattaaagcaagataggctattaagtgcagagggagagaaaatgcctccaacatgtgaggaagtaatgagagaaatcatagaattttaaggccatgatttaaggccatcatggccttaatcttccgcttcctcgctcactgactcgctgcgctcggtcgttcggctgcggcgagcggtatcagctcactcaaaggcggtaatacggttatccacagaatcaggggataacgcaggaaagaacatgtgagcaaaaggccagcaaaaggccaggaaccgtaaaaaggccgcgttgctggcgtttttccataggctccgcccccctgacgagcatcacaaaaatcgacgctcaagtcagaggtggcgaaacccgacaggactataaagataccaggcgtttccccctggaagctccctcgtgcgctctcctgttccgaccctgccgcttaccggatacctgtccgcctttctcccttcgggaagcgtggcgctttctcatagctcacgctgtaggtatctcagttcggtgtaggtcgttcgctccaagctgggctgtgtgcacgaaccccccgttcagcccgaccgctgcgccttatccggtaactatcgtcttgagtccaacccggtaagacacgacttatcgccactggcagcagccactggtaacaggattagcagagcgaggtatgtaggcggtgctacagagttcttgaagtggtggcctaactacggctacactagaagaacagtatttggtatctgcgctctgctgaagccagttaccttcggaaaaagagttggtagctcttgatccggcaaacaaaccaccgctggtagcggtggtttttttgtttgcaagcagcagattacgcgcagaaaaaaaggatctcaagaagatcctttgatcttttctacggggtctgacgctcagtggaacgaaaactcacgttaagggattttggtcatgagattatcaaaaaggatcttcacctagatccttttaaattaaaaatgaagttttaaatcaatctaaagtatatatgagtaaacttggtctgacagttaccaatgcttaatcagtgaggcacctatctcagcgatctgtctatttcgttcatccatagttgcctgactcggggggggggggcgctgaggtctgcctcgtgaagaaggtgttgctgactcataccaggcctgaatcgccccatcatccagccagaaagtgagggagccacggttgatgagagctttgttgtaggtggaccagttggtgattttgaacttttgctttgccacggaacggtctgcgttgtcgggaagatgcgtgatctgatccttcaactcagcaaaagttcgatttattcaacaaagccgccgtcccgtcaagtcagcgtaatgctctgccagtgttacaaccaattaaccaattctgattagaaaaactcatcgagcatcaaatgaaactgcaatttattcatatcaggattatcaataccatatttttgaaaaagccgtttctgtaatgaaggagaaaactcaccgaggcagttccataggatggcaagatcctggtatcggtctgcgattccgactcgtccaacatcaatacaacctattaatttcccctcgtcaaaaataaggttatcaagtgagaaatcaccatgagtgacgactgaatccggtgagaatggcaaaagcttatgcatttctttccagacttgttcaacaggccagccattacgctcgtcatcaaaatcactcgcatcaaccaaaccgttattcattcgtgattgcgcctgagcgagacgaaatacgcgatcgctgttaaaaggacaattacaaacaggaatcgaatgcaaccggcgcaggaacactgccagcgcatcaacaatattttcacctgaatcaggatattcttctaatacctggaatgctgttttcccggggatcgcagtggtgagtaaccatgcatcatcaggagtacggataaaatgcttgatggtcggaagaggcataaattccgtcagccagtttagtctgaccatctcatctgtaacatcattggcaacgctacctttgccatgtttcagaaacaactctggcgcatcgggcttcccatacaatcgatagattgtcgcacctgattgcccgacattatcgcgagcccatttatacccatataaatcagcatccatgttggaatttaatcgcggcctcgagcaagacgtttcccgttgaatatggctcataacaccccttgtattactgtttatgtaagcagacagttttattgttcatgatgatatatttttatcttgtgcaatgtaacatcagagattttgagacacaacgtggctttccccccccccccattattgaagcatttatcagggttattgtctcatgagcggatacatatttgaatgtatttagaaaaataaacaaataggggttccgcgcacatttccccgaaaagtgccacctgacgtctaagaaaccattattatcatgacattaacctataaaaataggcgtatcacgaggccctttcgtc

SEQ ID NO: 117 - protein, 472 aa, Homo sapiens
MGWSCIILFLVATATGVHSQLQLQESGPGVVKPSETLSLTCTISGGSFSTYYWTWIRQPPGKGLEWVGYIGNGGRSLNYNPSLKSRITLSVDASKNQFSLKVTSVTAADTAVYYCGRARGLRGNWFDVWGPGVLVTVSSASTKGPSVFPLAPSSRSTSESTAALGCLVKDYFPEPVTVSWNSGSLTSGVHTFPAVLQSSGLYSLSSVVTVPSSSLGTQTYVCNVNHKPSNTKVDKRVEIKTCGGGSKPPTCPPCTSPELLGGPSVFLFPPKPKDTLMISRTPEVTCVVVDVSQEDPDVKFNWYVNGAEVHHAQTKPRETQYNSTYRVVSVLTVTHQDWLNGKEYTCKVSNKALPAPIQKTISKDKGQPREPQVYTLPPSREELTKNQVSLTCLVKGFYPSDIVVEWESSGQPENTYKTTPPVLDSDGSYFLYSKLTVDKSRWQQGNVFSCSVMHEALHNHYTQKSLSLSPGK

SEQ ID NO: 118 - DNA, 5118 bp, Homo sapiens
  source 1..5118: mol_type = genomic DNA
tcgcgcgtttcggtgatgacggtgaaaacctctgacacatgcagctcccggagacggtcacagcttgtctgtaagcggatgccgggagcagacaagcccgtcagggcgcgtcagcgggtgttggcgggtgtcggggctggcttaactatgcggcatcagagcagattgtactgagagtgcaccatatgcggtgtgaaataccgcacagatgcgtaaggagaaaataccgcatcagattggctattggccattgcatacgttgtatccatatcataatatgtacatttatattggctcatgtccaacattaccgccatgttgacattgattattgactagttattaatagtaatcaattacggggtcattagttcatagcccatatatggagttccgcgttacataacttacggtaaatggcccgcctggctgaccgcccaacgacccccgcccattgacgtcaataatgacgtatgttcccatagtaacgccaatagggactttccattgacgtcaatgggtggagtatttacggtaaactgcccacttggcagtacatcaagtgtatcatatgccaagtacgccccctattgacgtcaatgacggtaaatggcccgcctggcattatgcccagtacatgaccttatgggactttcctacttggcagtacatctacgtattagtcatcgctattaccatggtgatgcggttttggcagtacatcaatgggcgtggatagcggtttgactcacggggatttccaagtctccaccccattgacgtcaatgggagtttgttttggcaccaaaatcaacgggactttccaaaatgtcgtaacaactccgccccattgacgcaaatgggcggtaggcgtgtacggtgggaggtctatataagcagagctcgtttagtgaaccgtcagatcgcctggagacgccatccacgctgttttgacctccatagaagacaccgggaccgatccagcctccatcggctcgcatctctccttcacgcgcccgccgccctacctgaggccgccatccacgccggttgagtcgcgttctgccgcctcccgcctgtggtgcctcctgaactgcgtccgccgtctaggtaagtttaaagctcaggtcgagaccgggcctttgtccggcgctcccttggagcctacctagactcagccggctctccacgctttgcctgaccctgcttgctcaactctagttaacggtggagggcagtgtagtctgagcagtacacgttgctgccgcgcgcgccaccagacataatagctgacagactaacagactgttcctttccatgggtcttttctgcagtcaccgtcgtcgacacgtgtgatcagatatcgcggccgctctagaccaccatgggatggtcatgtatcatcctttttctagtagcaactgcaaccggtgtacattcccaggctgccctgactcagcctccctctgtgtctgggtctcctggacagtcggtcaccatctcctgcactggaaccagcagtgacatcggtggttataactatgtctcctggtaccaacaacacccaggcaaagcccccaaagtcatgatttatgaggtcagtaagcggccctcaggggtctctgatcgcttctctggttccaaatctggcaacatagcctccctgaccatctctgggctccaggctgaggacgaggctgattattactgcagctcatatgcaggcagcaacactttcttattcggaggagggacccggctgacagtactaggtcagcccaaggctgccccctcggtcactctcttcccgccctcctctgaggagcttcaagccaacaaggccacactagtgtgtctgatcagtgacttctacccgggagccgtggaagtggcctggaaggcagatggcagcgctgtcaacgcgggagtggagaccaccaaaccctccaaacagagcaacaacaagtacgcggccagcagctacctgagcctgacgtccgaccagtggaagtcccacaagagctacagctgccaggtcacgcacgaagggagcaccgtggagaagacagtggcccctgcagaatgttcatagggatccagatctgctgtgccttctagttgccagccatctgttgtttgcccctcccccgtgccttccttgaccctggaaggtgccactcccactgtcctttcctaataaaatgaggaaattgcatcgcattgtctgagtaggtgtcattctattctggggggtggggtggggcaggacagcaagggggaggattgggaagacaatagcaggcatgctggggatgcggtgggctctatgggtacccaggtgctgaagaattgacccggttcctcctgggccagaaagaagcaggcacatccccttctctgtgacacaccctgtccacgcccctggttcttagttccagccccactcataggacactcatagctcaggagggctccgccttcaatcccacccgctaaagtacatggagcggtctctccctccctcatcagcccaccaaaccaaacctagcctccaagagtgggaagaaattaaagcaagataggctattaagtgcagagggagagaaaatgcctccaacatgtgaggaagtaatgagagaaatcatagaattttaaggccatgatttaaggccatcatggccttaatcttccgcttcctcgctcactgactcgctgcgctcggtcgttcggctgcggcgagcggtatcagctcactcaaaggcggtaatacggttatccacagaatcaggggataacgcaggaaagaacatgtgagcaaaaggccagcaaaaggccaggaaccgtaaaaaggccgcgttgctggcgtttttccataggctccgcccccctgacgagcatcacaaaaatcgacgctcaagtcagaggtggcgaaacccgacaggactataaagataccaggcgtttccccctggaagctccctcgtgcgctctcctgttccgaccctgccgcttaccggatacctgtccgcctttctcccttcgggaagcgtggcgctttctcatagctcacgctgtaggtatctcagttcggtgtaggtcgttcgctccaagctgggctgtgtgcacgaaccccccgttcagcccgaccgctgcgccttatccggtaactatcgtcttgagtccaacccggtaagacacgacttatcgccactggcagcagccactggtaacaggattagcagagcgaggtatgtaggcggtgctacagagttcttgaagtggtggcctaactacggctacactagaagaacagtatttggtatctgcgctctgctgaagccagttaccttcggaaaaagagttggtagctcttgatccggcaaacaaaccaccgctggtagcggtggtttttttgtttgcaagcagcagattacgcgcagaaaaaaaggatctcaagaagatcctttgatcttttctacggggtctgacgctcagtggaacgaaaactcacgttaagggattttggtcatgagattatcaaaaaggatcttcacctagatccttttaaattaaaaatgaagttttaaatcaatctaaagtatatatgagtaaacttggtctgacagttaccaatgcttaatcagtgaggcacctatctcagcgatctgtctatttcgttcatccatagttgcctgactcggggggggggggcgctgaggtctgcctcgtgaagaaggtgttgctgactcataccaggcctgaatcgccccatcatccagccagaaagtgagggagccacggttgatgagagctttgttgtaggtggaccagttggtgattttgaacttttgctttgccacggaacggtctgcgttgtcgggaagatgcgtgatctgatccttcaactcagcaaaagttcgatttattcaacaaagccgccgtcccgtcaagtcagcgtaatgctctgccagtgttacaaccaattaaccaattctgattagaaaaactcatcgagcatcaaatgaaactgcaatttattcatatcaggattatcaataccatatttttgaaaaagccgtttctgtaatgaaggagaaaactcaccgaggcagttccataggatggcaagatcctggtatcggtctgcgattccgactcgtccaacatcaatacaacctattaatttcccctcgtcaaaaataaggttatcaagtgagaaatcaccatgagtgacgactgaatccggtgagaatggcaaaagcttatgcatttctttccagacttgttcaacaggccagccattacgctcgtcatcaaaatcactcgcatcaaccaaaccgttattcattcgtgattgcgcctgagcgagacgaaatacgcgatcgctgttaaaaggacaattacaaacaggaatcgaatgcaaccggcgcaggaacactgccagcgcatcaacaatattttcacctgaatcaggatattcttctaatacctggaatgctgttttcccggggatcgcagtggtgagtaaccatgcatcatcaggagtacggataaaatgcttgatggtcggaagaggcataaattccgtcagccagtttagtctgaccatctcatctgtaacatcattggcaacgctacctttgccatgtttcagaaacaactctggcgcatcgggcttcccatacaatcgatagattgtcgcacctgattgcccgacattatcgcgagcccatttatacccatataaatcagcatccatgttggaatttaatcgcggcctcgagcaagacgtttcccgttgaatatggctcataacaccccttgtattactgtttatgtaagcagacagttttattgttcatgatgatatatttttatcttgtgcaatgtaacatcagagattttgagacacaacgtggctttccccccccccccattattgaagcatttatcagggttattgtctcatgagcggatacatatttgaatgtatttagaaaaataaacaaataggggttccgcgcacatttccccgaaaagtgccacctgacgtctaagaaaccattattatcatgacattaacctataaaaataggcgtatcacgaggccctttcgtc

SEQ ID NO: 119 - protein, 235 aa, Homo sapiens
MGWSCIILFLVATATGVHSQAALTQPPSVSGSPGQSVTISCTGTSSDIGGYNYVSWYQQHPGKAPKVMIYEVSKRPSGVSDRFSGSKSGNIASLTISGLQAEDEADYYCSSYAGSNTFLFGGGTRLTVLGQPKAAPSVTLFPPSSEELQANKATLVCLISDFYPGAVEVAWKADGSAVNAGVETTKPSKQSNNKYAASSYLSLTSDQWKSHKSYSCQVTHEGSTVEKTVAPAECS

SEQ ID NO: 120 - DNA, 5823 bp, Homo sapiens
  source 1..5823: mol_type = genomic DNA
tcgcgcgtttcggtgatgacggtgaaaacctctgacacatgcagctcccggagacggtcacagcttgtctgtaagcggatgccgggagcagacaagcccgtcagggcgcgtcagcgggtgttggcgggtgtcggggctggcttaactatgcggcatcagagcagattgtactgagagtgcaccatatgcggtgtgaaataccgcacagatgcgtaaggagaaaataccgcatcagattggctattggccattgcatacgttgtatccatatcataatatgtacatttatattggctcatgtccaacattaccgccatgttgacattgattattgactagttattaatagtaatcaattacggggtcattagttcatagcccatatatggagttccgcgttacataacttacggtaaatggcccgcctggctgaccgcccaacgacccccgcccattgacgtcaataatgacgtatgttcccatagtaacgccaatagggactttccattgacgtcaatgggtggagtatttacggtaaactgcccacttggcagtacatcaagtgtatcatatgccaagtacgccccctattgacgtcaatgacggtaaatggcccgcctggcattatgcccagtacatgaccttatgggactttcctacttggcagtacatctacgtattagtcatcgctattaccatggtgatgcggttttggcagtacatcaatgggcgtggatagcggtttgactcacggggatttccaagtctccaccccattgacgtcaatgggagtttgttttggcaccaaaatcaacgggactttccaaaatgtcgtaacaactccgccccattgacgcaaatgggcggtaggcgtgtacggtgggaggtctatataagcagagctcgtttagtgaaccgtcagatcgcctggagacgccatccacgctgttttgacctccatagaagacaccgggaccgatccagcctccatcggctcgcatctctccttcacgcgcccgccgccctacctgaggccgccatccacgccggttgagtcgcgttctgccgcctcccgcctgtggtgcctcctgaactgcgtccgccgtctaggtaagtttaaagctcaggtcgagaccgggcctttgtccggcgctcccttggagcctacctagactcagccggctctccacgctttgcctgaccctgcttgctcaactctagttaacggtggagggcagtgtagtctgagcagtactcgttgctgccgcgcgcgccaccagacataatagctgacagactaacagactgttcctttccatgggtcttttctgcagtcaccgtcgtcgacacgtgtgatcagatatcgcggccgctctagaccaccatgggatggtcatgtatcatcctttttctagtagcaactgcaaccggtgtacattcccaactgcagttgcaggagtcgggcccaggagtggtgaagccttcggagaccctgtccctcacctgcactatctctggtggctccttcagtacttactactggacctggattcgccagcccccagggaagggactggagtgggttgggtatatcggtaatggtggtcgtagcctcaactacaacccctccctcaagagtcgcatcaccctgtcagtagacgcgtccaagaaccagttctccctgaaggtgacctctgtgaccgccgcggacacggccgtctattactgtgggagagccaggggactccgcggaaactggttcgatgtctggggcccgggagtcctggtcaccgtctcctcagctagcaccaagggcccatcggtcttccccctggcaccctcctccaagagcacctctgggggcacagcggccctgggctgcctggtcaaggactacttccccgaaccggtgacggtgtcgtggaactcaggcgccctgaccagcggcgtgcacaccttcccggctgtcctacagtcctcaggactctactccctcagcagcgtggtgaccgtgccctccagcagcttgggcacccagacctacatctgcaacgtgaatcacaagcccagcaacaccaaggtggacaagaaagttgagcccaaatcttgtgacaaaactcacacatgcccaccgtgcccagcacctgaactcctggggggaccgtcagtcttcctcttccccccaaaacccaaggacaccctcatgatctcccggacccctgaggtcacatgcgtggtggtggacgtgagccacgaagaccctgaggtcaagttcaactggtacgtggacggcgtggaggtgcataatgccaagacaaagccgcgggaggagcagtacaacagcacgtaccgtgtggtcagcgtcctcaccgtcctgcaccaggactggctgaatggcaaggagtacaagtgcaaggtctccaacaaagccctcccagcccccatcgagaaaaccatctccaaagccaaagggcagccccgagaaccacaggtgtacaccctgcccccatcccgggatgagctgaccaagaaccaggtcagcctgacctgcctggtcaaaggcttctatcccagcgacatcgccgtggagtgggagagcaatgggcagccggagaacaactacaagaccacgcctcccgtgctggactccgacggctccttcttcctctacagcaagctcaccgtggacaagagcaggtggcagcaggggaacgtcttctcatgctccgtgatgcatgaggctctgcacaaccactacacgcagaagagcctctccctgtctccgggtaaatgatgaggatccagatctgctgtgccttctagttgccagccatctgttgtttgcccctcccccgtgccttccttgaccctggaaggtgccactcccactgtcctttcctaataaaatgaggaaattgcatcgcattgtctgagtaggtgtcattctattctggggggtggggtggggcaggacagcaagggggaggattgggaagacaatagcaggcatgctggggatgcggtgggctctatgggtacccaggtgctgaagaattgacccggttcctcctgggccagaaagaagcaggcacatccccttctctgtgacacaccctgtccacgcccctggttcttagttccagccccactcataggacactcatagctcaggagggctccgccttcaatcccacccgctaaagtacttggagcggtctctccctccctcatcagcccaccaaaccaaacctagcctccaagagtgggaagaaattaaagcaagataggctattaagtgcagagggagagaaaatgcctccaacatgtgaggaagtaatgagagaaatcatagaattttaaggccatgatttaaggccatcatggccttaatcttccgcttcctcgctcactgactcgctgcgctcggtcgttcggctgcggcgagcggtatcagctcactcaaaggcggtaatacggttatccacagaatcaggggataacgcaggaaagaacatgtgagcaaaaggccagcaaaaggccaggaaccgtaaaaaggccgcgttgctggcgtttttccataggctccgcccccctgacgagcatcacaaaaatcgacgctcaagtcagaggtggcgaaacccgacaggactataaagataccaggcgtttccccctggaagctccctcgtgcgctctcctgttccgaccctgccgcttaccggatacctgtccgcctttctcccttcgggaagcgtggcgctttctcatagctcacgctgtaggtatctcagttcggtgtaggtcgttcgctccaagctgggctgtgtgcacgaaccccccgttcagcccgaccgctgcgccttatccggtaactatcgtcttgagtccaacccggtaagacacgacttatcgccactggcagcagccactggtaacaggattagcagagcgaggtatgtaggcggtgctacagagttcttgaagtggtggcctaactacggctacactagaagaacagtatttggtatctgcgctctgctgaagccagttaccttcggaaaaagagttggtagctcttgatccggcaaacaaaccaccgctggtagcggtggtttttttgtttgcaagcagcagattacgcgcagaaaaaaaggatctcaagaagatcctttgatcttttctacggggtctgacgctcagtggaacgaaaactcacgttaagggattttggtcatgagattatcaaaaaggatcttcacctagatccttttaaattaaaaatgaagttttaaatcaatctaaagtatatatgagtaaacttggtctgacagttaccaatgcttaatcagtgaggcacctatctcagcgatctgtctatttcgttcatccatagttgcctgactcggggggggggggcgctgaggtctgcctcgtgaagaaggtgttgctgactcataccaggcctgaatcgccccatcatccagccagaaagtgagggagccacggttgatgagagctttgttgtaggtggaccagttggtgattttgaacttttgctttgccacggaacggtctgcgttgtcgggaagatgcgtgatctgatccttcaactcagcaaaagttcgatttattcaacaaagccgccgtcccgtcaagtcagcgtaatgctctgccagtgttacaaccaattaaccaattctgattagaaaaactcatcgagcatcaaatgaaactgcaatttattcatatcaggattatcaataccatatttttgaaaaagccgtttctgtaatgaaggagaaaactcaccgaggcagttccataggatggcaagatcctggtatcggtctgcgattccgactcgtccaacatcaatacaacctattaatttcccctcgtcaaaaataaggttatcaagtgagaaatcaccatgagtgacgactgaatccggtgagaatggcaaaagcttatgcatttctttccagacttgttcaacaggccagccattacgctcgtcatcaaaatcactcgcatcaaccaaaccgttattcattcgtgattgcgcctgagcgagacgaaatacgcgatcgctgttaaaaggacaattacaaacaggaatcgaatgcaaccggcgcaggaacactgccagcgcatcaacaatattttcacctgaatcaggatattcttctaatacctggaatgctgttttcccggggatcgcagtggtgagtaaccatgcatcatcaggagtacggataaaatgcttgatggtcggaagaggcataaattccgtcagccagtttagtctgaccatctcatctgtaacatcattggcaacgctacctttgccatgtttcagaaacaactctggcgcatcgggcttcccatacaatcgatagattgtcgcacctgattgcccgacattatcgcgagcccatttatacccatataaatcagcatccatgttggaatttaatcgcggcctcgagcaagacgtttcccgttgaatatggctcataacaccccttgtattactgtttatgtaagcagacagttttattgttcatgatgatatatttttatcttgtgcaatgtaacatcagagattttgagacacaacgtggctttccccccccccccattattgaagcatttatcagggttattgtctcatgagcggatacatatttgaatgtatttagaaaaataaacaaataggggttccgcgcacatttccccgaaaagtgccacctgacgtctaagaaaccattattatcatgacattaacctataaaaataggcgtatcacgaggccctttcgtc

SEQ ID NO: 121 - protein, 469 aa, Homo sapiens
MGWSCIILFLVATATGVHSQLQLQESGPGVVKPSETLSLTCTISGGSFSTYYWTWIRQPPGKGLEWVGYIGNGGRSLNYNPSLKSRITLSVDASKNQFSLKVTSVTAADTAVYYCGRARGLRGNWFDVWGPGVLVTVSSASTKGPSVFPLAPSSKSTSGGTAALGCLVKDYFPEPVTVSWNSGALTSGVHTFPAVLQSSGLYSLSSVVTVPSSSLGTQTYICNVNHKPSNTKVDKKVEPKSCDKTHTCPPCPAPELLGGPSVFLFPPKPKDTLMISRTPEVTCVVVDVSHEDPEVKFNWYVDGVEVHNAKTKPREEQYNSTYRVVSVLTVLHQDWLNGKEYKCKVSNKALPAPIEKTISKAKGQPREPQVYTLPPSRDELTKNQVSLTCLVKGFYPSDIAVEWESNGQPENNYKTTPPVLDSDGSFFLYSKLTVDKSRWQQGNVFSCSVMHEALHNHYTQKSLSLSPGK

SEQ ID NO: 122 - DNA, 5118 bp, Homo sapiens
  source 1..5118: mol_type = genomic DNA
tcgcgcgtttcggtgatgacggtgaaaacctctgacacatgcagctcccggagacggtcacagcttgtctgtaagcggatgccgggagcagacaagcccgtcagggcgcgtcagcgggtgttggcgggtgtcggggctggcttaactatgcggcatcagagcagattgtactgagagtgcaccatatgcggtgtgaaataccgcacagatgcgtaaggagaaaataccgcatcagattggctattggccattgcatacgttgtatccatatcataatatgtacatttatattggctcatgtccaacattaccgccatgttgacattgattattgactagttattaatagtaatcaattacggggtcattagttcatagcccatatatggagttccgcgttacataacttacggtaaatggcccgcctggctgaccgcccaacgacccccgcccattgacgtcaataatgacgtatgttcccatagtaacgccaatagggactttccattgacgtcaatgggtggagtatttacggtaaactgcccacttggcagtacatcaagtgtatcatatgccaagtacgccccctattgacgtcaatgacggtaaatggcccgcctggcattatgcccagtacatgaccttatgggactttcctacttggcagtacatctacgtattagtcatcgctattaccatggtgatgcggttttggcagtacatcaatgggcgtggatagcggtttgactcacggggatttccaagtctccaccccattgacgtcaatgggagtttgttttggcaccaaaatcaacgggactttccaaaatgtcgtaacaactccgccccattgacgcaaatgggcggtaggcgtgtacggtgggaggtctatataagcagagctcgtttagtgaaccgtcagatcgcctggagacgccatccacgctgttttgacctccatagaagacaccgggaccgatccagcctccatcggctcgcatctctccttcacgcgcccgccgccctacctgaggccgccatccacgccggttgagtcgcgttctgccgcctcccgcctgtggtgcctcctgaactgcgtccgccgtctaggtaagtttaaagctcaggtcgagaccgggcctttgtccggcgctcccttggagcctacctagactcagccggctctccacgctttgcctgaccctgcttgctcaactctagttaacggtggagggcagtgtagtctgagcagtactcgttgctgccgcgcgcgccaccagacataatagctgacagactaacagactgttcctttccatgggtcttttctgcagtcaccgtcgtcgacacgtgtgatcagatatcgcggccgctctagaccaccatgggatggtcatgtatcatcctttttctagtagcaactgcaaccggtgtacattcccaggctgccctgactcagcctccctctgtgtctgggtctcctggacagtcggtcaccatctcctgcactggaaccagcagtgacatcggtggttataactatgtctcctggtaccaacaacacccaggcaaagcccccaaagtcatgatttatgaggtcagtaagcggccctcaggggtctctgatcgcttctctggttccaaatctggcaacatagcctccctgaccatctctgggctccaggctgaggacgaggctgattattactgcagctcatatgcaggcagcaacactttcttattcggaggagggacccggctgacagtcctaggtcagcccaaggctgccccctcggtcactctgttcccgccctcctctgaggagcttcaagccaacaaggccacactggtgtgtctcataagtgacttctacccgggagccgtgacagtggcctggaaggcagatagcagccccgtcaaggcgggagtggagaccaccacaccctccaaacaaagcaacaacaagtacgcggccagcagctatctgagcctgacgcctgagcagtggaagtcccacagaagctacagctgccaggtcacgcatgaagggagcaccgtggagaagacagtggcccctacagaatgttcatgaggatccagatctgctgtgccttctagttgccagccatctgttgtttgcccctcccccgtgccttccttgaccctggaaggtgccactcccactgtcctttcctaataaaatgaggaaattgcatcgcattgtctgagtaggtgtcattctattctggggggtggggtggggcaggacagcaagggggaggattgggaagacaatagcaggcatgctggggatgcggtgggctctatgggtacccaggtgctgaagaattgacccggttcctcctgggccagaaagaagcaggcacatccccttctctgtgacacaccctgtccacgcccctggttcttagttccagccccactcataggacactcatagctcaggagggctccgccttcaatcccacccgctaaagtacttggagcggtctctccctccctcatcagcccaccaaaccaaacctagcctccaagagtgggaagaaattaaagcaagataggctattaagtgcagagggagagaaaatgcctccaacatgtgaggaagtaatgagagaaatcatagaattttaaggccatgatttaaggccatcatggccttaatcttccgcttcctcgctcactgactcgctgcgctcggtcgttcggctgcggcgagcggtatcagctcactcaaaggcggtaatacggttatccacagaatcaggggataacgcaggaaagaacatgtgagcaaaaggccagcaaaaggccaggaaccgtaaaaaggccgcgttgctggcgtttttccataggctccgcccccctgacgagcatcacaaaaatcgacgctcaagtcagaggtggcgaaacccgacaggactataaagataccaggcgtttccccctggaagctccctcgtgcgctctcctgttccgaccctgccgcttaccggatacctgtccgcctttctcccttcgggaagcgtggcgctttctcatagctcacgctgtaggtatctcagttcggtgtaggtcgttcgctccaagctgggctgtgtgcacgaaccccccgttcagcccgaccgctgcgccttatccggtaactatcgtcttgagtccaacccggtaagacacgacttatcgccactggcagcagccactggtaacaggattagcagagcgaggtatgtaggcggtgctacagagttcttgaagtggtggcctaactacggctacactagaagaacagtatttggtatctgcgctctgctgaagccagttaccttcggaaaaagagttggtagctcttgatccggcaaacaaaccaccgctggtagcggtggtttttttgtttgcaagcagcagattacgcgcagaaaaaaaggatctcaagaagatcctttgatcttttctacggggtctgacgctcagtggaacgaaaactcacgttaagggattttggtcatgagattatcaaaaaggatcttcacctagatccttttaaattaaaaatgaagttttaaatcaatctaaagtatatatgagtaaacttggtctgacagttaccaatgcttaatcagtgaggcacctatctcagcgatctgtctatttcgttcatccatagttgcctgactcggggggggggggcgctgaggtctgcctcgtgaagaaggtgttgctgactcataccaggcctgaatcgccccatcatccagccagaaagtgagggagccacggttgatgagagctttgttgtaggtggaccagttggtgattttgaacttttgctttgccacggaacggtctgcgttgtcgggaagatgcgtgatctgatccttcaactcagcaaaagttcgatttattcaacaaagccgccgtcccgtcaagtcagcgtaatgctctgccagtgttacaaccaattaaccaattctgattagaaaaactcatcgagcatcaaatgaaactgcaatttattcatatcaggattatcaataccatatttttgaaaaagccgtttctgtaatgaaggagaaaactcaccgaggcagttccataggatggcaagatcctggtatcggtctgcgattccgactcgtccaacatcaatacaacctattaatttcccctcgtcaaaaataaggttatcaagtgagaaatcaccatgagtgacgactgaatccggtgagaatggcaaaagcttatgcatttctttccagacttgttcaacaggccagccattacgctcgtcatcaaaatcactcgcatcaaccaaaccgttattcattcgtgattgcgcctgagcgagacgaaatacgcgatcgctgttaaaaggacaattacaaacaggaatcgaatgcaaccggcgcaggaacactgccagcgcatcaacaatattttcacctgaatcaggatattcttctaatacctggaatgctgttttcccggggatcgcagtggtgagtaaccatgcatcatcaggagtacggataaaatgcttgatggtcggaagaggcataaattccgtcagccagtttagtctgaccatctcatctgtaacatcattggcaacgctacctttgccatgtttcagaaacaactctggcgcatcgggcttcccatacaatcgatagattgtcgcacctgattgcccgacattatcgcgagcccatttatacccatataaatcagcatccatgttggaatttaatcgcggcctcgagcaagacgtttcccgttgaatatggctcataacaccccttgtattactgtttatgtaagcagacagttttattgttcatgatgatatatttttatcttgtgcaatgtaacatcagagattttgagacacaacgtggctttccccccccccccattattgaagcatttatcagggttattgtctcatgagcggatacatatttgaatgtatttagaaaaataaacaaataggggttccgcgcacatttccccgaaaagtgccacctgacgtctaagaaaccattattatcatgacattaacctataaaaataggcgtatcacgaggccctttcgtc

SEQ ID NO: 123 - protein, 235 aa, Homo sapiens
MGWSCIILFLVATATGVHSQAALTQPPSVSGSPGQSVTISCTGTSSDIGGYNYVSWYQQHPGKAPKVMIYEVSKRPSGVSDRFSGSKSGNIASLTISGLQAEDEADYYCSSYAGSNTFLFGGGTRLTVLGQPKAAPSVTLFPPSSEELQANKATLVCLISDFYPGAVTVAWKADSSPVKAGVETTTPSKQSNNKYAASSYLSLTPEQWKSHRSYSCQVTHEGSTVEKTVAPTECS

SEQ ID NO: 124 - protein, 907 aa, Homo sapiens
MEAALLVCQYTIQSLIHLTGEDPGFFNVEIPEFPFYPTCNVCTADVNVTINFDVGGKKHQLDLDFGQLTPHTKAVYQPRGAFGGSENATNLFLLELLGAGELALTMRSKKLPINVTTGEEQQVSLESVDVYFQDVFGTMWCHHAEMQNPVYLIPETVPYIKWDNCNSTNITAVVRAQGLDVTLPLSLPTSAQDSNFSVKTEMLGNEIDIECIMEDGEISQVLPGDNKFNITCSGYESHVPSGGILTSTSPVATPIPGTGYAYSLRLTPRPVSRFLGNNSILYVFYSGNGPKASGGDYCIQSNIVFSDEIPASQDMPTNTTDITYVGDNATYSVPMVTSEDANSPNVTVTAFWAWPNNTETDFKCKWTLTSGTPSGCENISGAFASNRTFDITVSGLGTAPKTLIITRTATNATTTTHKVIFSKAPESTTTSPTSNTTGFAAPNTTTGLPSSTHVPTNLTAPASTGPTVSTADVTSPTPAGTTSGASPVTPSPSPRDNGTESKAPDMTSPTSAVTTPTPNATSPTSAVTTPTPNATSPTPAVTTPTPNATSPTLGKTSPTSAVTTPTPNATSPTLGKTSPTSAVTTPTPNATSPTLGKTSPTSAVTTPTPNATSPTVGETSPQANTTNHTLGGTSSTPVVTSPPKNATSAVTTGQHNITSSSTSSMSLRPSSISETLSPSTSDNSTSHMPLLTSAHPTGGENITQVTPASTSTHHVSTSSPAPRPGTTSQASGPGNSSTSTKPGEVNVTKGTPPKNATSPQAPSGQKTAVPTVTSTGGKANSTTGGKHTTGHGARTSTEPTTDYGGDSTTPRTRYNATTYLPPSTSSELRPRWTFTSPPVTTAQATVPVPPTSQPRFSNLSMLVLQWASLAVLTLLLLLVMADCAFRRNLSTSHTYTTPPYDDAETYV

SEQ ID NO: 125 - protein, 426 aa, Homo sapiens
EAALLVCQYTIQSLIHLTGEDPGFFNVEIPEFPFYPTCNVCTADVNVTINFDVGGKKHQLDLDFGQLTPHTKAVYQPRGAFGGSENATNLFLLELLGAGELALTMRSKKLPINVTTGEEQQVSLESVDVYFQDVFGTMWCHHAEMQNPVYLIPETVPYIKWDNCNSTNITAVVRAQGLDVTLPLSLPTSAQDSNFSVKTEMLGNEIDIECIMEDGEISQVLPGDNKFNITCSGYESHVPSGGILTSTSPVATPIPGTGYAYSLRLTPRPVSRFLGNNSILYVFYSGNGPKASGGDYCIQSNIVFSDEIPASQDMPTNTTDITYVGDNATYSVPMVTSEDANSPNVTVTAFWAWPNNTETDFKCKWTLTSGTPSGCENISGAFASNRTFDITVSGLGTAPKTLIITRTATNATTTTHKVIFSKAPGS

SEQ ID NO: 126 - DNA, 1281 bp, Homo sapiens
  source 1..1281: mol_type = genomic DNA
gaagctgccctgctcgtgtgccagtacaccatccagagcctgatccacctgaccggcgaggaccccggcttcttcaacgtggaaatccccgagttccccttctaccctacctgcaacgtgtgcaccgccgacgtgaacgtgaccatcaacttcgacgtgggcggcaagaagcaccagctggacctggatttcggccagctgacccctcacaccaaggccgtgtatcagcccagaggcgcctttggcggcagcgagaacgccaccaatctgtttctgctggaactcctaggcgccggcgagctggccctgaccatgagaagcaagaaactgcccatcaatgtgaccacaggcgaggaacagcaggtgtccctggaaagcgtggacgtgtactttcaagacgtgttcggcaccatgtggtgccaccacgccgagatgcagaaccccgtgtacctgatccccgagacagtgccctacatcaagtgggacaactgcaacagcaccaacatcaccgccgtcgtgcgggcccagggactggatgtgacactgcctctgagcctgcctaccagcgcccaggacagcaacttcagcgtgaaaaccgagatgctgggcaacgagatcgacatcgagtgcatcatggaagatggcgagatcagccaggtgctgcccggcgacaacaagttcaacatcacatgcagcggctacgagagccacgtgccatctggcggcatcctgaccagcacaagcccagtggccacacccatccctggcacaggctacgcctacagcctgagactgacccccagacccgtgtccagattcctgggcaacaacagcatcctgtacgtgttctacagcggcaacggccccaaggcctctggcggcgattactgtatccagagcaacatcgtgttcagcgacgagatccccgccagccaggacatgcccaccaataccaccgacatcacgtacgtgggcgacaatgccacctacagcgtgccaatggtcacctccgaggacgccaacagccccaacgtgaccgtgacagccttttgggcctggcctaacaacaccgagacagacttcaagtgcaagtggaccctgacctccggcacccctagcggctgcgagaatatcagcggagccttcgccagcaaccggaccttcgatatcaccgtgtctggcctgggcaccgcccccaagaccctgatcatcaccagaaccgccacaaatgccaccaccacaacccacaaagtgatcttcagcaaggcccccggctctggc

SEQ ID NO: 127 - protein, 426 aa, Homo sapiens
EAALLVCQYTIQSLIHLTGEDPGFFNVEIPEFPFYPTCNVCTADVNVTINFDVGGKKHQLDLDFGQLTPHTKAVYQPRGAFGGSENATNLFLLELLGAGELALTMRSKKLPINVTTGEEQNVSLESVDVYFQDVFGTMWCHHAEMQNPVYLIPETVPYIKWDNCNSTNITAVVRAQGLDVTLPLSLPTSAQDSNFSVKTEMLGNEIDIECIMEDGEISQVLPGDNKFNITCSGYESHVPSGGILTSTSPVATPIPGTGYAYSLRLTPRPVSRFLGNNSILYVFYSGNGPKASGGDYCIQSNIVFSDEIPASQDMPTNTTDITYVGDNATYSVPMVTSEDANSPNVTVTAFWAWPNNTETDFKCKWTLTSGTPSGCENISGAFASNRTFDITVSGLGTAPKTLIITRTATNATTTTHKVIFSKAPGS

SEQ ID NO: 128 - DNA, 1278 bp, Homo sapiens
  source 1..1278: mol_type = genomic DNA
gaagctgccctgctcgtgtgccagtacaccatccagagcctgatccacctgaccggcgaggaccccggcttcttcaacgtggaaatccccgagttccccttctaccctacctgcaacgtgtgcaccgccgacgtgaacgtgaccatcaacttcgacgtgggcggcaagaagcaccagctggacctggatttcggccagctgacccctcacaccaaggccgtgtatcagcccagaggcgcctttggcggcagcgagaacgccaccaatctgtttctgctggaactcctaggcgccggcgagctggccctgaccatgagaagcaagaaactgcccatcaatgtgaccacaggcgaggaacagaacgtgtccctggaaagcgtggacgtgtactttcaagacgtgttcggcaccatgtggtgccaccacgccgagatgcagaaccccgtgtacctgatccccgagacagtgccctacatcaagtgggacaactgcaacagcaccaacatcaccgccgtcgtgcgggcccagggactggatgtgacactgcctctgagcctgcctaccagcgcccaggacagcaacttcagcgtgaaaaccgagatgctgggcaacgagatcgacatcgagtgcatcatggaagatggcgagatcagccaggtgctgcccggcgacaacaagttcaacatcacatgcagcggctacgagagccacgtgccatctggcggcatcctgaccagcacaagcccagtggccacacccatccctggcacaggctacgcctacagcctgagactgacccccagacccgtgtccagattcctgggcaacaacagcatcctgtacgtgttctacagcggcaacggccccaaggcctctggcggcgattactgtatccagagcaacatcgtgttcagcgacgagatccccgccagccaggacatgcccaccaataccaccgacatcacgtacgtgggcgacaatgccacctacagcgtgccaatggtcacctccgaggacgccaacagccccaacgtgaccgtgacagccttttgggcctggcctaacaacaccgagacagacttcaagtgcaagtggaccctgacctccggcacccctagcggctgcgagaatatcagcggagccttcgccagcaaccggaccttcgatatcaccgtgtctggcctgggcaccgcccccaagaccctgatcatcaccagaaccgccacaaatgccaccaccacaacccacaaagtgatcttcagcaaggcccccggctct

SEQ ID NO: 129 - protein, 427 aa, Homo sapiens
EAALLVCQYTIQSLIHLTGEDPGFFNVEIPEFPFYPTCNVCTADVNVTINFDVGGKKHQLDLDFGQLTPHTKAVYQPRGAFGGSENATNLFLLELLGAGELALTMRSKKLPINVTTGEEQQVSLESVDVYFQDVFGTMWCHHAEMQNPVYLIPETVPYIKWNNSCNSTNITAVVRAQGLDVTLPLSLPTSAQDSNFSVKTEMLGNEIDIECIMEDGEISQVLPGDNKFNITCSGYESHVPSGGILTSTSPVATPIPGTGYAYSLRLTPRPVSRFLGNNSILYVFYSGNGPKASGGDYCIQSNIVFSDEIPASQDMPTNTTDITYVGDNATYSVPMVTSEDANSPNVTVTAFWAWPNNTETDFKCKWTLTSGTPSGCENISGAFASNRTFDITVSGLGTAPKTLIITRTATNATTTTHKVIFSKAPGS

SEQ ID NO: 130 - DNA, 1281 bp, Homo sapiens
  source 1..1281: mol_type = genomic DNA
gaagctgccctgctcgtgtgccagtacaccatccagagcctgatccacctgaccggcgaggaccccggcttcttcaacgtggaaatccccgagttccccttctaccctacctgcaacgtgtgcaccgccgacgtgaacgtgaccatcaacttcgacgtgggcggcaagaagcaccagctggacctggatttcggccagctgacccctcacaccaaggccgtgtatcagcccagaggcgcctttggcggcagcgagaacgccaccaatctgtttctgctggaactcctaggcgccggcgagctggccctgaccatgagaagcaagaaactgcccatcaatgtgaccacaggcgaggaacagcaggtgtccctggaaagcgtggacgtgtactttcaagacgtgttcggcaccatgtggtgccaccacgccgagatgcagaaccccgtgtacctgatccccgagacagtgccctacatcaagtggaacaacagctgcaacagcaccaacatcaccgccgtcgtgcgggcccagggactggatgtgacactgcctctgagcctgcctaccagcgcccaggacagcaacttcagcgtgaaaaccgagatgctgggcaacgagatcgacatcgagtgcatcatggaagatggcgagatcagccaggtgctgcccggcgacaacaagttcaacatcacatgcagcggctacgagagccacgtgccatctggcggcatcctgaccagcacaagcccagtggccacacccatccctggcacaggctacgcctacagcctgagactgacccccagacccgtgtccagattcctgggcaacaacagcatcctgtacgtgttctacagcggcaacggccccaaggcctctggcggcgattactgtatccagagcaacatcgtgttcagcgacgagatccccgccagccaggacatgcccaccaataccaccgacatcacgtacgtgggcgacaatgccacctacagcgtgccaatggtcacctccgaggacgccaacagccccaacgtgaccgtgacagccttttgggcctggcctaacaacaccgagacagacttcaagtgcaagtggaccctgacctccggcacccctagcggctgcgagaatatcagcggagccttcgccagcaaccggaccttcgatatcaccgtgtctggcctgggcaccgcccccaagaccctgatcatcaccagaaccgccacaaatgccaccaccacaacccacaaagtgatcttcagcaaggcccccggctct

SEQ ID NO: 131 - protein, 426 aa, Homo sapiens
EAALLVCQYTIQSLIHLTGEDPGFFNVEIPEFPFYPTCNVCTADVNVTINFDVGGKKHQLDLDFGQLTPHTKAVYQPRGAFGGSENATNLFLLELLGAGELALTMRSKKLPINVTTGEEQQVSLESVDVYFQDVFGTMWCHHAEMQNPVYLIPETVPYIKWDNCNSTNITAVVRAQGLDVTLPLSLPTSAQDSNFSVKTEMLGNEIDIECIMEDGEISQVLPGDNKFNITCSGYESHVPSGGILTSTSPVATPIPGTGYAYSLRLTPRPVSRFLGNNSILYVFYSGNGPKASGGRYCIQSNIVFSDEIPASQDMPTNTTDITYVGDNATYSVPMVTSEDANSPNVTVTAFWAWPNNTETDFKCKWTLTSGTPSGCENISGAFASNRTFDITVSGLGTAPKTLIITRTATNATTTTHKVIFSKAPGS

SEQ ID NO: 132 - DNA, 1278 bp, Homo sapiens
  source 1..1278: mol_type = genomic DNA
gaagctgccctgctcgtgtgccagtacaccatccagagcctgatccacctgaccggcgaggaccccggcttcttcaacgtggaaatccccgagttccccttctaccctacctgcaacgtgtgcaccgccgacgtgaacgtgaccatcaacttcgacgtgggcggcaagaagcaccagctggacctggatttcggccagctgacccctcacaccaaggccgtgtatcagcccagaggcgcctttggcggcagcgagaacgccaccaatctgtttctgctggaactcctaggcgccggcgagctggccctgaccatgagaagcaagaaactgcccatcaatgtgaccacaggcgaggaacagcaggtgtccctggaaagcgtggacgtgtactttcaagacgtgttcggcaccatgtggtgccaccacgccgagatgcagaaccccgtgtacctgatccccgagacagtgccctacatcaagtgggacaactgcaacagcaccaacatcaccgccgtcgtgcgggcccagggactggatgtgacactgcctctgagcctgcctaccagcgcccaggacagcaacttcagcgtgaaaaccgagatgctgggcaacgagatcgacatcgagtgcatcatggaagatggcgagatcagccaggtgctgcccggcgacaacaagttcaacatcacatgcagcggctacgagagccacgtgccatctggcggcatcctgaccagcacaagcccagtggccacacccatccctggcacaggctacgcctacagcctgagactgacccccagacccgtgtccagattcctgggcaacaacagcatcctgtacgtgttctacagcggcaacggccccaaggcctctggcggccggtactgtatccagagcaacatcgtgttcagcgacgagatccccgccagccaggacatgcccaccaataccaccgacatcacgtacgtgggcgacaatgccacctacagcgtgccaatggtcacctccgaggacgccaacagccccaacgtgaccgtgacagccttttgggcctggcctaacaacaccgagacagacttcaagtgcaagtggaccctgacctccggcacccctagcggctgcgagaatatcagcggagccttcgccagcaaccggaccttcgatatcaccgtgtctggcctgggcaccgcccccaagaccctgatcatcaccagaaccgccacaaatgccaccaccacaacccacaaagtgatcttcagcaaggcccccggctct

SEQ ID NO: 133 - protein, 426 aa, Homo sapiens
EAALLVCQYTIQSLIHLTGEDPGFFNVEIPEFPFYPTCNVCTADVNVTINFDVGGKKHQLDLDFGQLTPHTKAVYQPRGAFGGSENATNLFLLELLGAGELALTMRSKKLPINVTTGEEQQVSLESVDVYFQDVFGTMWCHHAEMQNPVYLIPETVPYIKAAACNSTNITAVVRAQGLDVTLPLSLPTSAQDSNFSVKTEMLGNEIDIECIMEDGEISQVLPGDNKFNITCSGYESHVPSGGILTSTSPVATPIPGTGYAYSLRLTPRPVSRFLGNNSILYVFYSGNGPKASGGDYCIQSNIVFSDEIPASQDMPTNTTDITYVGDNATYSVPMVTSEDANSPNVTVTAFWAWPNNTETDFKCKWTLTSGTPSGCENISGAFASNRTFDITVSGLGTAPKTLIITRTATNATTTTHKVIFSKAPGS

SEQ ID NO: 134 - DNA, 1278 bp, Homo sapiens
  source 1..1278: mol_type = genomic DNA
gaagctgccctgctcgtgtgccagtacaccatccagagcctgatccacctgaccggcgaggaccccggcttcttcaacgtggaaatccccgagttccccttctaccctacctgcaacgtgtgcaccgccgacgtgaacgtgaccatcaacttcgacgtgggcggcaagaagcaccagctggacctggatttcggccagctgacccctcacaccaaggccgtgtatcagcccagaggcgcctttggcggcagcgagaacgccaccaatctgtttctgctggaactcctaggcgccggcgagctggccctgaccatgagaagcaagaaactgcccatcaatgtgaccacaggcgaggaacagcaggtgtccctggaaagcgtggacgtgtactttcaagacgtgttcggcaccatgtggtgccaccacgccgagatgcagaaccccgtgtacctgatccccgagacagtgccctacatcaaggccgccgcctgcaacagcaccaacatcaccgccgtcgtgcgggcccagggactggatgtgacactgcctctgagcctgcctaccagcgcccaggacagcaacttcagcgtgaaaaccgagatgctgggcaacgagatcgacatcgagtgcatcatggaagatggcgagatcagccaggtgctgcccggcgacaacaagttcaacatcacatgcagcggctacgagagccacgtgccatctggcggcatcctgaccagcacaagcccagtggccacacccatccctggcacaggctacgcctacagcctgagactgacccccagacccgtgtccagattcctgggcaacaacagcatcctgtacgtgttctacagcggcaacggccccaaggcctctggcggcgattactgtatccagagcaacatcgtgttcagcgacgagatccccgccagccaggacatgcccaccaataccaccgacatcacgtacgtgggcgacaatgccacctacagcgtgccaatggtcacctccgaggacgccaacagccccaacgtgaccgtgacagccttttgggcctggcctaacaacaccgagacagacttcaagtgcaagtggaccctgacctccggcacccctagcggctgcgagaatatcagcggagccttcgccagcaaccggaccttcgatatcaccgtgtctggcctgggcaccgcccccaagaccctgatcatcaccagaaccgccacaaatgccaccaccacaacccacaaagtgatcttcagcaaggcccccggctct

SEQ ID NO: 135 - protein, 426 aa, Homo sapiens
EAALLVCQYTIQSLIHLTGEDPGFFNVEIPEFPFYPTCNVCTADVNVTINFDVGGKKHQLDLDFGQLTPHTKAVYQPRGAFGGSENATNLFLLELLGAGELALTMRSKKLPINVTTGEEQQVSLESVDVYFQDVFGTMWCHHAEMQNPVYLIPETVPYRKWDNCNSTNITAVVRAQGLDVTLPLSLPTSAQDSNFSVKTEMLGNEIDIECIMEDGEISQVLPGDNKFNITCSGYESHVPSGGILTSTSPVATPIPGTGYAYSLRLTPRPVSRFLGNNSILYVFYSGNGPKASGGRYCIQSNIVFSDEIPASQDMPTNTTDITYVGDNATYSVPMVTSEDANSPNVTVTAFWAWPNNTETDFKCKWTLTSGTPSGCENISGAFASNRTFDITVSGLGTAPKTLIITRTATNATTTTHKVIFSKAPGS

SEQ ID NO: 136 - DNA, 1278 bp, Homo sapiens
  source 1..1278: mol_type = genomic DNA
gaagctgccctgctcgtgtgccagtacaccatccagagcctgatccacctgaccggcgaggaccccggcttcttcaacgtggaaatccccgagttccccttctaccctacctgcaacgtgtgcaccgccgacgtgaacgtgaccatcaacttcgacgtgggcggcaagaagcaccagctggacctggatttcggccagctgacccctcacaccaaggccgtgtatcagcccagaggcgcctttggcggcagcgagaacgccaccaatctgtttctgctggaactcctaggcgccggcgagctggccctgaccatgagaagcaagaaactgcccatcaatgtgaccacaggcgaggaacagcaggtgtccctggaaagcgtggacgtgtactttcaagacgtgttcggcaccatgtggtgccaccacgccgagatgcagaaccccgtgtacctgatccccgagacagtgccctaccggaagtgggacaactgcaacagcaccaacatcaccgccgtcgtgcgggcccagggactggatgtgacactgcctctgagcctgcctaccagcgcccaggacagcaacttcagcgtgaaaaccgagatgctgggcaacgagatcgacatcgagtgcatcatggaagatggcgagatcagccaggtgctgcccggcgacaacaagttcaacatcacatgcagcggctacgagagccacgtgccatctggcggcatcctgaccagcacaagcccagtggccacacccatccctggcacaggctacgcctacagcctgagactgacccccagacccgtgtccagattcctgggcaacaacagcatcctgtacgtgttctacagcggcaacggccccaaggcctctggcggccggtactgtatccagagcaacatcgtgttcagcgacgagatccccgccagccaggacatgcccaccaataccaccgacatcacgtacgtgggcgacaatgccacctacagcgtgccaatggtcacctccgaggacgccaacagccccaacgtgaccgtgacagccttttgggcctggcctaacaacaccgagacagacttcaagtgcaagtggaccctgacctccggcacccctagcggctgcgagaatatcagcggagccttcgccagcaaccggaccttcgatatcaccgtgtctggcctgggcaccgcccccaagaccctgatcatcaccagaaccgccacaaatgccaccaccacaacccacaaagtgatcttcagcaaggcccccggctct

SEQ ID NO: 137 - protein, 426 aa, Homo sapiens
EAALLVCQYTIQSLIHLTGEDPGFFNVEIPEFPFYPTCNVCTADVNVTINFDVGGKKHQLDLDFGQLTPHTKAVYQPRGAFGGSENATNLFLLELLGAGELALTMRSKKLPINVTTGEEQQVSLESVDVYFQDVFGTMWCHHAEMQNPVYLIPETVRYIKWDNCNSTNITAVVRAQGLDVTLPLSLPTSAQDSNFSVKTEMLGNEIDIECIMEDGEISQVLPGDNKFNITCSGYESHVPSGGILTSTSPVATPIPGTGYAYSLRLTPRPVSRFLGNNSILYVFYSGNGPKASGGRYCIQSNIVFSDEIPASQDMPTNTTDITYVGDNATYSVPMVTSEDANSPNVTVTAFWAWPNNTETDFKCKWTLTSGTPSGCENISGAFASNRTFDITVSGLGTAPKTLIITRTATNATTTTHKVIFSKAPGS

SEQ ID NO: 138 - DNA, 1278 bp, Homo sapiens
  source 1..1278: mol_type = genomic DNA
gaagctgccctgctcgtgtgccagtacaccatccagagcctgatccacctgaccggcgaggaccccggcttcttcaacgtggaaatccccgagttccccttctaccctacctgcaacgtgtgcaccgccgacgtgaacgtgaccatcaacttcgacgtgggcggcaagaagcaccagctggacctggatttcggccagctgacccctcacaccaaggccgtgtatcagcccagaggcgcctttggcggcagcgagaacgccaccaatctgtttctgctggaactcctaggcgccggcgagctggccctgaccatgagaagcaagaaactgcccatcaatgtgaccacaggcgaggaacagcaggtgtccctggaaagcgtggacgtgtactttcaagacgtgttcggcaccatgtggtgccaccacgccgagatgcagaaccccgtgtacctgatccccgagacagtgcggtacatcaagtgggacaactgcaacagcaccaacatcaccgccgtcgtgcgggcccagggactggatgtgacactgcctctgagcctgcctaccagcgcccaggacagcaacttcagcgtgaaaaccgagatgctgggcaacgagatcgacatcgagtgcatcatggaagatggcgagatcagccaggtgctgcccggcgacaacaagttcaacatcacatgcagcggctacgagagccacgtgccatctggcggcatcctgaccagcacaagcccagtggccacacccatccctggcacaggctacgcctacagcctgagactgacccccagacccgtgtccagattcctgggcaacaacagcatcctgtacgtgttctacagcggcaacggccccaaggcctctggcggccggtactgtatccagagcaacatcgtgttcagcgacgagatccccgccagccaggacatgcccaccaataccaccgacatcacgtacgtgggcgacaatgccacctacagcgtgccaatggtcacctccgaggacgccaacagccccaacgtgaccgtgacagccttttgggcctggcctaacaacaccgagacagacttcaagtgcaagtggaccctgacctccggcacccctagcggctgcgagaatatcagcggagccttcgccagcaaccggaccttcgatatcaccgtgtctggcctgggcaccgcccccaagaccctgatcatcaccagaaccgccacaaatgccaccaccacaacccacaaagtgatcttcagcaaggcccccggctct

SEQ ID NO: 139 - protein, 426 aa, Homo sapiens
EAALLVCQYTIQSLIHLTGEDPGFFNVEIPEFPFYPTCNVCTADVNVTINFDVGGKKHQLDLDFGQLTPHTKAVYQPRGAFGGSENATNLFLLELLGAGELALTMRSKKLPINVTTGEEQQVSLESVDVYFQDVFGTMWCHHAEMQNPVYLIPETVNYTKWDNCNSTNITAVVRAQGLDVTLPLSLPTSAQDSNFSVKTEMLGNEIDIECIMEDGEISQVLPGDNKFNITCSGYESHVPSGGILTSTSPVATPIPGTGYAYSLRLTPRPVSRFLGNNSILYVFYSGNGPKASGGRYCIQSNIVFSDEIPASQDMPTNTTDITYVGDNATYSVPMVTSEDANSPNVTVTAFWAWPNNTETDFKCKWTLTSGTPSGCENISGAFASNRTFDITVSGLGTAPKTLIITRTATNATTTTHKVIFSKAPGS

SEQ ID NO: 140 - DNA, 1278 bp, Homo sapiens
  source 1..1278: mol_type = genomic DNA
gaagctgccctgctcgtgtgccagtacaccatccagagcctgatccacctgaccggcgaggaccccggcttcttcaacgtggaaatccccgagttccccttctaccctacctgcaacgtgtgcaccgccgacgtgaacgtgaccatcaacttcgacgtgggcggcaagaagcaccagctggacctggatttcggccagctgacccctcacaccaaggccgtgtatcagcccagaggcgcctttggcggcagcgagaacgccaccaatctgtttctgctggaactcctaggcgccggcgagctggccctgaccatgagaagcaagaaactgcccatcaatgtgaccacaggcgaggaacagcaggtgtccctggaaagcgtggacgtgtactttcaagacgtgttcggcaccatgtggtgccaccacgccgagatgcagaaccccgtgtacctgatccccgagacagtgaactacaccaagtgggacaactgcaacagcaccaacatcaccgccgtcgtgcgggcccagggactggatgtgacactgcctctgagcctgcctaccagcgcccaggacagcaacttcagcgtgaaaaccgagatgctgggcaacgagatcgacatcgagtgcatcatggaagatggcgagatcagccaggtgctgcccggcgacaacaagttcaacatcacatgcagcggctacgagagccacgtgccatctggcggcatcctgaccagcacaagcccagtggccacacccatccctggcacaggctacgcctacagcctgagactgacccccagacccgtgtccagattcctgggcaacaacagcatcctgtacgtgttctacagcggcaacggccccaaggcctctggcggccggtactgtatccagagcaacatcgtgttcagcgacgagatccccgccagccaggacatgcccaccaataccaccgacatcacgtacgtgggcgacaatgccacctacagcgtgccaatggtcacctccgaggacgccaacagccccaacgtgaccgtgacagccttttgggcctggcctaacaacaccgagacagacttcaagtgcaagtggaccctgacctccggcacccctagcggctgcgagaatatcagcggagccttcgccagcaaccggaccttcgatatcaccgtgtctggcctgggcaccgcccccaagaccctgatcatcaccagaaccgccacaaatgccaccaccacaacccacaaagtgatcttcagcaaggcccccggctct

SEQ ID NO: 141 - protein, 426 aa, Homo sapiens
EAALLVCQYTIQSLIHLTGEDPGFFNVEIPEFPFYPTCNVCTADVNVTINFDVGGKKHQLDLDFGQLTPHTKAVYQPRGAFGGSENATNLFLLELLGAGELALTMRSKKLPINVTTGEEQQVSLESVDVYFQDVFGTMWCHHAEMQNPVYLIPETVRYRKWDNCNSTNITAVVRAQGLDVTLPLSLPTSAQDSNFSVKTEMLGNEIDIECIMEDGEISQVLPGDNKFNITCSGYESHVPSGGILTSTSPVATPIPGTGYAYSLRLTPRPVSRFLGNNSILYVFYSGNGPKASGGRYCIQSNIVFSDEIPASQDMPTNTTDITYVGDNATYSVPMVTSEDANSPNVTVTAFWAWPNNTETDFKCKWTLTSGTPSGCENISGAFASNRTFDITVSGLGTAPKTLIITRTATNATTTTHKVIFSKAPGS

SEQ ID NO: 142 - DNA, 1278 bp, Homo sapiens
  source 1..1278: mol_type = genomic DNA
gaagctgccctgctcgtgtgccagtacaccatccagagcctgatccacctgaccggcgaggaccccggcttcttcaacgtggaaatccccgagttccccttctaccctacctgcaacgtgtgcaccgccgacgtgaacgtgaccatcaacttcgacgtgggcggcaagaagcaccagctggacctggatttcggccagctgacccctcacaccaaggccgtgtatcagcccagaggcgcctttggcggcagcgagaacgccaccaatctgtttctgctggaactcctaggcgccggcgagctggccctgaccatgagaagcaagaaactgcccatcaatgtgaccacaggcgaggaacagcaggtgtccctggaaagcgtggacgtgtactttcaagacgtgttcggcaccatgtggtgccaccacgccgagatgcagaaccccgtgtacctgatccccgagacagtgcggtaccggaagtgggacaactgcaacagcaccaacatcaccgccgtcgtgcgggcccagggactggatgtgacactgcctctgagcctgcctaccagcgcccaggacagcaacttcagcgtgaaaaccgagatgctgggcaacgagatcgacatcgagtgcatcatggaagatggcgagatcagccaggtgctgcccggcgacaacaagttcaacatcacatgcagcggctacgagagccacgtgccatctggcggcatcctgaccagcacaagcccagtggccacacccatccctggcacaggctacgcctacagcctgagactgacccccagacccgtgtccagattcctgggcaacaacagcatcctgtacgtgttctacagcggcaacggccccaaggcctctggcggccggtactgtatccagagcaacatcgtgttcagcgacgagatccccgccagccaggacatgcccaccaataccaccgacatcacgtacgtgggcgacaatgccacctacagcgtgccaatggtcacctccgaggacgccaacagccccaacgtgaccgtgacagccttttgggcctggcctaacaacaccgagacagacttcaagtgcaagtggaccctgacctccggcacccctagcggctgcgagaatatcagcggagccttcgccagcaaccggaccttcgatatcaccgtgtctggcctgggcaccgcccccaagaccctgatcatcaccagaaccgccacaaatgccaccaccacaacccacaaagtgatcttcagcaaggcccccggctct

SEQ ID NO: 143 - protein, 447 aa, Homo sapiens
EAALLVCQYTIQSLIHLTGEDPGFFNVEIPEFPFYPTCNVCTADVNVTINFDVGGKKHQLDLDFGQLTPHTKAVYQPRGAFGGSENATNLFLLELLGAGELALTMRSKKLPINVTTGEEQQVSLESVDVYFQDVFGTMWCHHAEMQNPVYLIPETVPYIKWDNCNSTNITAVVRAQGLDVTLPLSLPTSAQDSNFSVKTEMLGNEIDIECIMEDGEISQVLPGDNKFNITCSGYESHVPSGGILTSTSPVATPIPGTGYAYSLRLTPRPVSRFLGNNSILYVFYSGNGPKASGGDYCIQSNIVFSDEIPASQDMPTNTTDITYVGDNATYSVPMVTSEDANSPNVTVTAFWAWPNNTETDFKCKWTLTSGTPSGCENISGAFASNRTFDITVSGLGTAPKTLIITRTATNATTTTHKVIFSKAPGSGLNDIFEAQKIEWHEHHHHHH

SEQ ID NO: 144 - DNA, 1341 bp, Homo sapiens
  source 1..1341: mol_type = genomic DNA
gaagctgccctgctcgtgtgccagtacaccatccagagcctgatccacctgaccggcgaggaccccggcttcttcaacgtggaaatccccgagttccccttctaccctacctgcaacgtgtgcaccgccgacgtgaacgtgaccatcaacttcgacgtgggcggcaagaagcaccagctggacctggatttcggccagctgacccctcacaccaaggccgtgtatcagcccagaggcgcctttggcggcagcgagaacgccaccaatctgtttctgctggaactcctaggcgccggcgagctggccctgaccatgagaagcaagaaactgcccatcaatgtgaccacaggcgaggaacagcaggtgtccctggaaagcgtggacgtgtactttcaagacgtgttcggcaccatgtggtgccaccacgccgagatgcagaaccccgtgtacctgatccccgagacagtgccctacatcaagtgggacaactgcaacagcaccaacatcaccgccgtcgtgcgggcccagggactggatgtgacactgcctctgagcctgcctaccagcgcccaggacagcaacttcagcgtgaaaaccgagatgctgggcaacgagatcgacatcgagtgcatcatggaagatggcgagatcagccaggtgctgcccggcgacaacaagttcaacatcacatgcagcggctacgagagccacgtgccatctggcggcatcctgaccagcacaagcccagtggccacacccatccctggcacaggctacgcctacagcctgagactgacccccagacccgtgtccagattcctgggcaacaacagcatcctgtacgtgttctacagcggcaacggccccaaggcctctggcggcgattactgtatccagagcaacatcgtgttcagcgacgagatccccgccagccaggacatgcccaccaataccaccgacatcacgtacgtgggcgacaatgccacctacagcgtgccaatggtcacctccgaggacgccaacagccccaacgtgaccgtgacagccttttgggcctggcctaacaacaccgagacagacttcaagtgcaagtggaccctgacctccggcacccctagcggctgcgagaatatcagcggagccttcgccagcaaccggaccttcgatatcaccgtgtctggcctgggcaccgcccccaagaccctgatcatcaccagaaccgccacaaatgccaccaccacaacccacaaagtgatcttcagcaaggcccccggctctggcctgaacgacatttttgaggcccagaagattgagtggcatgaacatcaccaccaccaccat

SEQ ID NO: 145 - protein, 447 aa, Homo sapiens
EAALLVCQYTIQSLIHLTGEDPGFFNVEIPEFPFYPTCNVCTADVNVTINFDVGGKKHQLDLDFGQLTPHTKAVYQPRGAFGGSENATNLFLLELLGAGELALTMRSKKLPINVTTGEEQNVSLESVDVYFQDVFGTMWCHHAEMQNPVYLIPETVPYIKWDNCNSTNITAVVRAQGLDVTLPLSLPTSAQDSNFSVKTEMLGNEIDIECIMEDGEISQVLPGDNKFNITCSGYESHVPSGGILTSTSPVATPIPGTGYAYSLRLTPRPVSRFLGNNSILYVFYSGNGPKASGGDYCIQSNIVFSDEIPASQDMPTNTTDITYVGDNATYSVPMVTSEDANSPNVTVTAFWAWPNNTETDFKCKWTLTSGTPSGCENISGAFASNRTFDITVSGLGTAPKTLIITRTATNATTTTHKVIFSKAPGSGLNDIFEAQKIEWHEHHHHHH

SEQ ID NO: 146 - DNA, 1341 bp, Homo sapiens
  source 1..1341: mol_type = genomic DNA
gaagctgccctgctcgtgtgccagtacaccatccagagcctgatccacctgaccggcgaggaccccggcttcttcaacgtggaaatccccgagttccccttctaccctacctgcaacgtgtgcaccgccgacgtgaacgtgaccatcaacttcgacgtgggcggcaagaagcaccagctggacctggatttcggccagctgacccctcacaccaaggccgtgtatcagcccagaggcgcctttggcggcagcgagaacgccaccaatctgtttctgctggaactcctaggcgccggcgagctggccctgaccatgagaagcaagaaactgcccatcaatgtgaccacaggcgaggaacagaacgtgtccctggaaagcgtggacgtgtactttcaagacgtgttcggcaccatgtggtgccaccacgccgagatgcagaaccccgtgtacctgatccccgagacagtgccctacatcaagtgggacaactgcaacagcaccaacatcaccgccgtcgtgcgggcccagggactggatgtgacactgcctctgagcctgcctaccagcgcccaggacagcaacttcagcgtgaaaaccgagatgctgggcaacgagatcgacatcgagtgcatcatggaagatggcgagatcagccaggtgctgcccggcgacaacaagttcaacatcacatgcagcggctacgagagccacgtgccatctggcggcatcctgaccagcacaagcccagtggccacacccatccctggcacaggctacgcctacagcctgagactgacccccagacccgtgtccagattcctgggcaacaacagcatcctgtacgtgttctacagcggcaacggccccaaggcctctggcggcgattactgtatccagagcaacatcgtgttcagcgacgagatccccgccagccaggacatgcccaccaataccaccgacatcacgtacgtgggcgacaatgccacctacagcgtgccaatggtcacctccgaggacgccaacagccccaacgtgaccgtgacagccttttgggcctggcctaacaacaccgagacagacttcaagtgcaagtggaccctgacctccggcacccctagcggctgcgagaatatcagcggagccttcgccagcaaccggaccttcgatatcaccgtgtctggcctgggcaccgcccccaagaccctgatcatcaccagaaccgccacaaatgccaccaccacaacccacaaagtgatcttcagcaaggcccccggctctggcctgaacgacatttttgaggcccagaagattgagtggcatgaacatcaccaccaccaccat

SEQ ID NO: 147 - protein, 448 aa, Homo sapiens
EAALLVCQYTIQSLIHLTGEDPGFFNVEIPEFPFYPTCNVCTADVNVTINFDVGGKKHQLDLDFGQLTPHTKAVYQPRGAFGGSENATNLFLLELLGAGELALTMRSKKLPINVTTGEEQQVSLESVDVYFQDVFGTMWCHHAEMQNPVYLIPETVPYIKWNNSCNSTNITAVVRAQGLDVTLPLSLPTSAQDSNFSVKTEMLGNEIDIECIMEDGEISQVLPGDNKFNITCSGYESHVPSGGILTSTSPVATPIPGTGYAYSLRLTPRPVSRFLGNNSILYVFYSGNGPKASGGDYCIQSNIVFSDEIPASQDMPTNTTDITYVGDNATYSVPMVTSEDANSPNVTVTAFWAWPNNTETDFKCKWTLTSGTPSGCENISGAFASNRTFDITVSGLGTAPKTLIITRTATNATTTTHKVIFSKAPGSGLNDIFEAQKIEWHEHHHHHH

SEQ ID NO: 148 - DNA, 1344 bp, Homo sapiens
  source 1..1344: mol_type = genomic DNA
gaagctgccctgctcgtgtgccagtacaccatccagagcctgatccacctgaccggcgaggaccccggcttcttcaacgtggaaatccccgagttccccttctaccctacctgcaacgtgtgcaccgccgacgtgaacgtgaccatcaacttcgacgtgggcggcaagaagcaccagctggacctggatttcggccagctgacccctcacaccaaggccgtgtatcagcccagaggcgcctttggcggcagcgagaacgccaccaatctgtttctgctggaactcctaggcgccggcgagctggccctgaccatgagaagcaagaaactgcccatcaatgtgaccacaggcgaggaacagcaggtgtccctggaaagcgtggacgtgtactttcaagacgtgttcggcaccatgtggtgccaccacgccgagatgcagaaccccgtgtacctgatccccgagacagtgccctacatcaagtggaacaacagctgcaacagcaccaacatcaccgccgtcgtgcgggcccagggactggatgtgacactgcctctgagcctgcctaccagcgcccaggacagcaacttcagcgtgaaaaccgagatgctgggcaacgagatcgacatcgagtgcatcatggaagatggcgagatcagccaggtgctgcccggcgacaacaagttcaacatcacatgcagcggctacgagagccacgtgccatctggcggcatcctgaccagcacaagcccagtggccacacccatccctggcacaggctacgcctacagcctgagactgacccccagacccgtgtccagattcctgggcaacaacagcatcctgtacgtgttctacagcggcaacggccccaaggcctctggcggcgattactgtatccagagcaacatcgtgttcagcgacgagatccccgccagccaggacatgcccaccaataccaccgacatcacgtacgtgggcgacaatgccacctacagcgtgccaatggtcacctccgaggacgccaacagccccaacgtgaccgtgacagccttttgggcctggcctaacaacaccgagacagacttcaagtgcaagtggaccctgacctccggcacccctagcggctgcgagaatatcagcggagccttcgccagcaaccggaccttcgatatcaccgtgtctggcctgggcaccgcccccaagaccctgatcatcaccagaaccgccacaaatgccaccaccacaacccacaaagtgatcttcagcaaggcccccggctctggcctgaacgacatttttgaggcccagaagattgagtggcatgaacatcaccaccaccaccat

SEQ ID NO: 149 - protein, 447 aa, Homo sapiens
EAALLVCQYTIQSLIHLTGEDPGFFNVEIPEFPFYPTCNVCTADVNVTINFDVGGKKHQLDLDFGQLTPHTKAVYQPRGAFGGSENATNLFLLELLGAGELALTMRSKKLPINVTTGEEQQVSLESVDVYFQDVFGTMWCHHAEMQNPVYLIPETVPYIKWDNCNSTNITAVVRAQGLDVTLPLSLPTSAQDSNFSVKTEMLGNEIDIECIMEDGEISQVLPGDNKFNITCSGYESHVPSGGILTSTSPVATPIPGTGYAYSLRLTPRPVSRFLGNNSILYVFYSGNGPKASGGRYCIQSNIVFSDEIPASQDMPTNTTDITYVGDNATYSVPMVTSEDANSPNVTVTAFWAWPNNTETDFKCKWTLTSGTPSGCENISGAFASNRTFDITVSGLGTAPKTLIITRTATNATTTTHKVIFSKAPGSGLNDIFEAQKIEWHEHHHHHH

SEQ ID NO: 150 - DNA, 1341 bp, Homo sapiens
  source 1..1341: mol_type = genomic DNA
gaagctgccctgctcgtgtgccagtacaccatccagagcctgatccacctgaccggcgaggaccccggcttcttcaacgtggaaatccccgagttccccttctaccctacctgcaacgtgtgcaccgccgacgtgaacgtgaccatcaacttcgacgtgggcggcaagaagcaccagctggacctggatttcggccagctgacccctcacaccaaggccgtgtatcagcccagaggcgcctttggcggcagcgagaacgccaccaatctgtttctgctggaactcctaggcgccggcgagctggccctgaccatgagaagcaagaaactgcccatcaatgtgaccacaggcgaggaacagcaggtgtccctggaaagcgtggacgtgtactttcaagacgtgttcggcaccatgtggtgccaccacgccgagatgcagaaccccgtgtacctgatccccgagacagtgccctacatcaagtgggacaactgcaacagcaccaacatcaccgccgtcgtgcgggcccagggactggatgtgacactgcctctgagcctgcctaccagcgcccaggacagcaacttcagcgtgaaaaccgagatgctgggcaacgagatcgacatcgagtgcatcatggaagatggcgagatcagccaggtgctgcccggcgacaacaagttcaacatcacatgcagcggctacgagagccacgtgccatctggcggcatcctgaccagcacaagcccagtggccacacccatccctggcacaggctacgcctacagcctgagactgacccccagacccgtgtccagattcctgggcaacaacagcatcctgtacgtgttctacagcggcaacggccccaaggcctctggcggccggtactgtatccagagcaacatcgtgttcagcgacgagatccccgccagccaggacatgcccaccaataccaccgacatcacgtacgtgggcgacaatgccacctacagcgtgccaatggtcacctccgaggacgccaacagccccaacgtgaccgtgacagccttttgggcctggcctaacaacaccgagacagacttcaagtgcaagtggaccctgacctccggcacccctagcggctgcgagaatatcagcggagccttcgccagcaaccggaccttcgatatcaccgtgtctggcctgggcaccgcccccaagaccctgatcatcaccagaaccgccacaaatgccaccaccacaacccacaaagtgatcttcagcaaggcccccggctctggcctgaacgacatttttgaggcccagaagattgagtggcatgaacatcaccaccaccaccat

SEQ ID NO: 151 - protein, 447 aa, Homo sapiens
EAALLVCQYTIQSLIHLTGEDPGFFNVEIPEFPFYPTCNVCTADVNVTINFDVGGKKHQLDLDFGQLTPHTKAVYQPRGAFGGSENATNLFLLELLGAGELALTMRSKKLPINVTTGEEQQVSLESVDVYFQDVFGTMWCHHAEMQNPVYLIPETVPYIKAAACNSTNITAVVRAQGLDVTLPLSLPTSAQDSNFSVKTEMLGNEIDIECIMEDGEISQVLPGDNKFNITCSGYESHVPSGGILTSTSPVATPIPGTGYAYSLRLTPRPVSRFLGNNSILYVFYSGNGPKASGGDYCIQSNIVFSDEIPASQDMPTNTTDITYVGDNATYSVPMVTSEDANSPNVTVTAFWAWPNNTETDFKCKWTLTSGTPSGCENISGAFASNRTFDITVSGLGTAPKTLIITRTATNATTTTHKVIFSKAPGSGLNDIFEAQKIEWHEHHHHHH

SEQ ID NO: 152 - DNA, 1341 bp, Homo sapiens
  source 1..1341: mol_type = genomic DNA
gaagctgccctgctcgtgtgccagtacaccatccagagcctgatccacctgaccggcgaggaccccggcttcttcaacgtggaaatccccgagttccccttctaccctacctgcaacgtgtgcaccgccgacgtgaacgtgaccatcaacttcgacgtgggcggcaagaagcaccagctggacctggatttcggccagctgacccctcacaccaaggccgtgtatcagcccagaggcgcctttggcggcagcgagaacgccaccaatctgtttctgctggaactcctaggcgccggcgagctggccctgaccatgagaagcaagaaactgcccatcaatgtgaccacaggcgaggaacagcaggtgtccctggaaagcgtggacgtgtactttcaagacgtgttcggcaccatgtggtgccaccacgccgagatgcagaaccccgtgtacctgatccccgagacagtgccctacatcaaggccgccgcctgcaacagcaccaacatcaccgccgtcgtgcgggcccagggactggatgtgacactgcctctgagcctgcctaccagcgcccaggacagcaacttcagcgtgaaaaccgagatgctgggcaacgagatcgacatcgagtgcatcatggaagatggcgagatcagccaggtgctgcccggcgacaacaagttcaacatcacatgcagcggctacgagagccacgtgccatctggcggcatcctgaccagcacaagcccagtggccacacccatccctggcacaggctacgcctacagcctgagactgacccccagacccgtgtccagattcctgggcaacaacagcatcctgtacgtgttctacagcggcaacggccccaaggcctctggcggcgattactgtatccagagcaacatcgtgttcagcgacgagatccccgccagccaggacatgcccaccaataccaccgacatcacgtacgtgggcgacaatgccacctacagcgtgccaatggtcacctccgaggacgccaacagccccaacgtgaccgtgacagccttttgggcctggcctaacaacaccgagacagacttcaagtgcaagtggaccctgacctccggcacccctagcggctgcgagaatatcagcggagccttcgccagcaaccggaccttcgatatcaccgtgtctggcctgggcaccgcccccaagaccctgatcatcaccagaaccgccacaaatgccaccaccacaacccacaaagtgatcttcagcaaggcccccggctctggcctgaacgacatttttgaggcccagaagattgagtggcatgaacatcaccaccaccaccat

SEQ ID NO: 153 - protein, 447 aa, Homo sapiens
EAALLVCQYTIQSLIHLTGEDPGFFNVEIPEFPFYPTCNVCTADVNVTINFDVGGKKHQLDLDFGQLTPHTKAVYQPRGAFGGSENATNLFLLELLGAGELALTMRSKKLPINVTTGEEQQVSLESVDVYFQDVFGTMWCHHAEMQNPVYLIPETVPYRKWDNCNSTNITAVVRAQGLDVTLPLSLPTSAQDSNFSVKTEMLGNEIDIECIMEDGEISQVLPGDNKFNITCSGYESHVPSGGILTSTSPVATPIPGTGYAYSLRLTPRPVSRFLGNNSILYVFYSGNGPKASGGRYCIQSNIVFSDEIPASQDMPTNTTDITYVGDNATYSVPMVTSEDANSPNVTVTAFWAWPNNTETDFKCKWTLTSGTPSGCENISGAFASNRTFDITVSGLGTAPKTLIITRTATNATTTTHKVIFSKAPGSGLNDIFEAQKIEWHEHHHHHH

SEQ ID NO: 154 - DNA, 1341 bp, Homo sapiens
  source 1..1341: mol_type = genomic DNA
gaagctgccctgctcgtgtgccagtacaccatccagagcctgatccacctgaccggcgaggaccccggcttcttcaacgtggaaatccccgagttccccttctaccctacctgcaacgtgtgcaccgccgacgtgaacgtgaccatcaacttcgacgtgggcggcaagaagcaccagctggacctggatttcggccagctgacccctcacaccaaggccgtgtatcagcccagaggcgcctttggcggcagcgagaacgccaccaatctgtttctgctggaactcctaggcgccggcgagctggccctgaccatgagaagcaagaaactgcccatcaatgtgaccacaggcgaggaacagcaggtgtccctggaaagcgtggacgtgtactttcaagacgtgttcggcaccatgtggtgccaccacgccgagatgcagaaccccgtgtacctgatccccgagacagtgccctaccggaagtgggacaactgcaacagcaccaacatcaccgccgtcgtgcgggcccagggactggatgtgacactgcctctgagcctgcctaccagcgcccaggacagcaacttcagcgtgaaaaccgagatgctgggcaacgagatcgacatcgagtgcatcatggaagatggcgagatcagccaggtgctgcccggcgacaacaagttcaacatcacatgcagcggctacgagagccacgtgccatctggcggcatcctgaccagcacaagcccagtggccacacccatccctggcacaggctacgcctacagcctgagactgacccccagacccgtgtccagattcctgggcaacaacagcatcctgtacgtgttctacagcggcaacggccccaaggcctctggcggccggtactgtatccagagcaacatcgtgttcagcgacgagatccccgccagccaggacatgcccaccaataccaccgacatcacgtacgtgggcgacaatgccacctacagcgtgccaatggtcacctccgaggacgccaacagccccaacgtgaccgtgacagccttttgggcctggcctaacaacaccgagacagacttcaagtgcaagtggaccctgacctccggcacccctagcggctgcgagaatatcagcggagccttcgccagcaaccggaccttcgatatcaccgtgtctggcctgggcaccgcccccaagaccctgatcatcaccagaaccgccacaaatgccaccaccacaacccacaaagtgatcttcagcaaggcccccggctctggcctgaacgacatttttgaggcccagaagattgagtggcatgaacatcaccaccaccaccat

SEQ ID NO: 155 - protein, 447 aa, Homo sapiens
EAALLVCQYTIQSLIHLTGEDPGFFNVEIPEFPFYPTCNVCTADVNVTINFDVGGKKHQLDLDFGQLTPHTKAVYQPRGAFGGSENATNLFLLELLGAGELALTMRSKKLPINVTTGEEQQVSLESVDVYFQDVFGTMWCHHAEMQNPVYLIPETVRYIKWDNCNSTNITAVVRAQGLDVTLPLSLPTSAQDSNFSVKTEMLGNEIDIECIMEDGEISQVLPGDNKFNITCSGYESHVPSGGILTSTSPVATPIPGTGYAYSLRLTPRPVSRFLGNNSILYVFYSGNGPKASGGRYCIQSNIVFSDEIPASQDMPTNTTDITYVGDNATYSVPMVTSEDANSPNVTVTAFWAWPNNTETDFKCKWTLTSGTPSGCENISGAFASNRTFDITVSGLGTAPKTLIITRTATNATTTTHKVIFSKAPGSGLNDIFEAQKIEWHEHHHHHH

SEQ ID NO: 156 - DNA, 1341 bp, Homo sapiens
  source 1..1341: mol_type = genomic DNA
gaagctgccctgctcgtgtgccagtacaccatccagagcctgatccacctgaccggcgaggaccccggcttcttcaacgtggaaatccccgagttccccttctaccctacctgcaacgtgtgcaccgccgacgtgaacgtgaccatcaacttcgacgtgggcggcaagaagcaccagctggacctggatttcggccagctgacccctcacaccaaggccgtgtatcagcccagaggcgcctttggcggcagcgagaacgccaccaatctgtttctgctggaactcctaggcgccggcgagctggccctgaccatgagaagcaagaaactgcccatcaatgtgaccacaggcgaggaacagcaggtgtccctggaaagcgtggacgtgtactttcaagacgtgttcggcaccatgtggtgccaccacgccgagatgcagaaccccgtgtacctgatccccgagacagtgcggtacatcaagtgggacaactgcaacagcaccaacatcaccgccgtcgtgcgggcccagggactggatgtgacactgcctctgagcctgcctaccagcgcccaggacagcaacttcagcgtgaaaaccgagatgctgggcaacgagatcgacatcgagtgcatcatggaagatggcgagatcagccaggtgctgcccggcgacaacaagttcaacatcacatgcagcggctacgagagccacgtgccatctggcggcatcctgaccagcacaagcccagtggccacacccatccctggcacaggctacgcctacagcctgagactgacccccagacccgtgtccagattcctgggcaacaacagcatcctgtacgtgttctacagcggcaacggccccaaggcctctggcggccggtactgtatccagagcaacatcgtgttcagcgacgagatccccgccagccaggacatgcccaccaataccaccgacatcacgtacgtgggcgacaatgccacctacagcgtgccaatggtcacctccgaggacgccaacagccccaacgtgaccgtgacagccttttgggcctggcctaacaacaccgagacagacttcaagtgcaagtggaccctgacctccggcacccctagcggctgcgagaatatcagcggagccttcgccagcaaccggaccttcgatatcaccgtgtctggcctgggcaccgcccccaagaccctgatcatcaccagaaccgccacaaatgccaccaccacaacccacaaagtgatcttcagcaaggcccccggctctggcctgaacgacatttttgaggcccagaagattgagtggcatgaacatcaccaccaccaccat

SEQ ID NO: 157 - protein, 447 aa, Homo sapiens
EAALLVCQYTIQSLIHLTGEDPGFFNVEIPEFPFYPTCNVCTADVNVTINFDVGGKKHQLDLDFGQLTPHTKAVYQPRGAFGGSENATNLFLLELLGAGELALTMRSKKLPINVTTGEEQQVSLESVDVYFQDVFGTMWCHHAEMQNPVYLIPETVNYTKWDNCNSTNITAVVRAQGLDVTLPLSLPTSAQDSNFSVKTEMLGNEIDIECIMEDGEISQVLPGDNKFNITCSGYESHVPSGGILTSTSPVATPIPGTGYAYSLRLTPRPVSRFLGNNSILYVFYSGNGPKASGGRYCIQSNIVFSDEIPASQDMPTNTTDITYVGDNATYSVPMVTSEDANSPNVTVTAFWAWPNNTETDFKCKWTLTSGTPSGCENISGAFASNRTFDITVSGLGTAPKTLIITRTATNATTTTHKVIFSKAPGSGLNDIFEAQKIEWHEHHHHHH

SEQ ID NO: 158 - DNA, 1341 bp, Homo sapiens
  source 1..1341: mol_type = genomic DNA
gaagctgccctgctcgtgtgccagtacaccatccagagcctgatccacctgaccggcgaggaccccggcttcttcaacgtggaaatccccgagttccccttctaccctacctgcaacgtgtgcaccgccgacgtgaacgtgaccatcaacttcgacgtgggcggcaagaagcaccagctggacctggatttcggccagctgacccctcacaccaaggccgtgtatcagcccagaggcgcctttggcggcagcgagaacgccaccaatctgtttctgctggaactcctaggcgccggcgagctggccctgaccatgagaagcaagaaactgcccatcaatgtgaccacaggcgaggaacagcaggtgtccctggaaagcgtggacgtgtactttcaagacgtgttcggcaccatgtggtgccaccacgccgagatgcagaaccccgtgtacctgatccccgagacagtgaactacaccaagtgggacaactgcaacagcaccaacatcaccgccgtcgtgcgggcccagggactggatgtgacactgcctctgagcctgcctaccagcgcccaggacagcaacttcagcgtgaaaaccgagatgctgggcaacgagatcgacatcgagtgcatcatggaagatggcgagatcagccaggtgctgcccggcgacaacaagttcaacatcacatgcagcggctacgagagccacgtgccatctggcggcatcctgaccagcacaagcccagtggccacacccatccctggcacaggctacgcctacagcctgagactgacccccagacccgtgtccagattcctgggcaacaacagcatcctgtacgtgttctacagcggcaacggccccaaggcctctggcggccggtactgtatccagagcaacatcgtgttcagcgacgagatccccgccagccaggacatgcccaccaataccaccgacatcacgtacgtgggcgacaatgccacctacagcgtgccaatggtcacctccgaggacgccaacagccccaacgtgaccgtgacagccttttgggcctggcctaacaacaccgagacagacttcaagtgcaagtggaccctgacctccggcacccctagcggctgcgagaatatcagcggagccttcgccagcaaccggaccttcgatatcaccgtgtctggcctgggcaccgcccccaagaccctgatcatcaccagaaccgccacaaatgccaccaccacaacccacaaagtgatcttcagcaaggcccccggctctggcctgaacgacatttttgaggcccagaagattgagtggcatgaacatcaccaccaccaccat

SEQ ID NO: 159 - protein, 447 aa, Homo sapiens
EAALLVCQYTIQSLIHLTGEDPGFFNVEIPEFPFYPTCNVCTADVNVTINFDVGGKKHQLDLDFGQLTPHTKAVYQPRGAFGGSENATNLFLLELLGAGELALTMRSKKLPINVTTGEEQQVSLESVDVYFQDVFGTMWCHHAEMQNPVYLIPETVRYRKWDNCNSTNITAVVRAQGLDVTLPLSLPTSAQDSNFSVKTEMLGNEIDIECIMEDGEISQVLPGDNKFNITCSGYESHVPSGGILTSTSPVATPIPGTGYAYSLRLTPRPVSRFLGNNSILYVFYSGNGPKASGGRYCIQSNIVFSDEIPASQDMPTNTTDITYVGDNATYSVPMVTSEDANSPNVTVTAFWAWPNNTETDFKCKWTLTSGTPSGCENISGAFASNRTFDITVSGLGTAPKTLIITRTATNATTTTHKVIFSKAPGSGLNDIFEAQKIEWHEHHHHHH

SEQ ID NO: 160 - DNA, 1341 bp, Homo sapiens
  source 1..1341: mol_type = genomic DNA
gaagctgccctgctcgtgtgccagtacaccatccagagcctgatccacctgaccggcgaggaccccggcttcttcaacgtggaaatccccgagttccccttctaccctacctgcaacgtgtgcaccgccgacgtgaacgtgaccatcaacttcgacgtgggcggcaagaagcaccagctggacctggatttcggccagctgacccctcacaccaaggccgtgtatcagcccagaggcgcctttggcggcagcgagaacgccaccaatctgtttctgctggaactcctaggcgccggcgagctggccctgaccatgagaagcaagaaactgcccatcaatgtgaccacaggcgaggaacagcaggtgtccctggaaagcgtggacgtgtactttcaagacgtgttcggcaccatgtggtgccaccacgccgagatgcagaaccccgtgtacctgatccccgagacagtgcggtaccggaagtgggacaactgcaacagcaccaacatcaccgccgtcgtgcgggcccagggactggatgtgacactgcctctgagcctgcctaccagcgcccaggacagcaacttcagcgtgaaaaccgagatgctgggcaacgagatcgacatcgagtgcatcatggaagatggcgagatcagccaggtgctgcccggcgacaacaagttcaacatcacatgcagcggctacgagagccacgtgccatctggcggcatcctgaccagcacaagcccagtggccacacccatccctggcacaggctacgcctacagcctgagactgacccccagacccgtgtccagattcctgggcaacaacagcatcctgtacgtgttctacagcggcaacggccccaaggcctctggcggccggtactgtatccagagcaacatcgtgttcagcgacgagatccccgccagccaggacatgcccaccaataccaccgacatcacgtacgtgggcgacaatgccacctacagcgtgccaatggtcacctccgaggacgccaacagccccaacgtgaccgtgacagccttttgggcctggcctaacaacaccgagacagacttcaagtgcaagtggaccctgacctccggcacccctagcggctgcgagaatatcagcggagccttcgccagcaaccggaccttcgatatcaccgtgtctggcctgggcaccgcccccaagaccctgatcatcaccagaaccgccacaaatgccaccaccacaacccacaaagtgatcttcagcaaggcccccggctctggcctgaacgacatttttgaggcccagaagattgagtggcatgaacatcaccaccaccaccat

SEQ ID NO: 161 - protein, 119 aa, Homo sapiens
QVQLVQSGADVRKPGASVKVSCKASTYIFTGYYIHWVRQAPGRGLEWLGWIHPNSGGTTYSQMFQGRVTMTRDRSITTSYMELSRLQSDDTAIYYCATLRFVEYSFDSWGQGTLVTVSS

SEQ ID NO: 162 - DNA, 357 bp, Homo sapiens
  source 1..357: mol_type = genomic DNA
caggtgcagctggtgcagtctggcgcagacgtgaggaagccaggagcctccgtgaaggtgtcttgtaaggccagcacctacatcttcacaggctactatatccactgggtgaggcaggcaccaggaaggggcctggagtggctgggctggattcaccctaactctggcggcaccacatacagccagatgtttcagggcagagtgaccatgacacgggacagatccatcaccacatcttatatggagctgagccggctgcagtccgacgataccgccatctactattgcgccacactgagattcgtggagtattcttttgatagctggggccagggcaccctggtgacagtgagctcc

SEQ ID NO: 163 - protein, 7 aa, Homo sapiens
TYIFTGY

SEQ ID NO: 164 - protein, 6 aa, Homo sapiens
HPNSGG

SEQ ID NO: 165 - protein, 10 aa, Homo sapiens
LRFVEYSFDS

SEQ ID NO: 166 - protein, 108 aa, Homo sapiens
EIVLTQSPGTLSLSPGERATLSCRASQSISSTYLAWYQQIPGQAPRLLIYGASSRAAGIPDRFSGGGSGTDFTLTISRLEPEDFAVYYCQQYGSSPRSFGQGTKLEIK

SEQ ID NO: 167 - DNA, 324 bp, Homo sapiens
  source 1..324: mol_type = genomic DNA
gagatcgtgctgacccagagcccaggcacactgagcctgtccccaggagagagggccaccctgtcctgtagagcctctcagagcatcagctccacatacctggcctggtatcagcagatcccaggacaggcacctaggctgctgatctacggagcctctagcagggcagcaggcatccccgaccgcttctccggcggaggctctggcaccgacttcaccctgacaatctctcggctggagcctgaggacttcgccgtgtactattgccagcagtatggctcctctccaaggtcctttggccagggcacaaagctggagatcaag

SEQ ID NO: 168 - protein, 12 aa, Homo sapiens
RASQSISSTYLA

SEQ ID NO: 169 - protein, 7 aa, Homo sapiens
GASSRAA

SEQ ID NO: 170 - protein, 9 aa, Homo sapiens
QQYGSSPRS

SEQ ID NO: 171 - protein, 119 aa, Homo sapiens
EVQLLESGGALVQPGGSLRLSCAASGFTFKTYAMSWVRQVPGKGLEWVSAISGSGTASYYADSVKGRFTLSRDNSKNTLYLQLSSLRDEDTGVYYCARRFLDWFGMDVWGLGTTVTVSS

SEQ ID NO: 172 - DNA, 357 bp, Homo sapiens
  source 1..357: mol_type = genomic DNA
gaggtgcagctgctggagagcggcggcgccctggtgcagccaggaggcagcctgcggctgtcctgtgccgcctctggcttcacctttaagacatacgccatgtcctgggtgaggcaggtgcctggcaagggcctggagtgggtgtctgccatctccggctctggcaccgcctcttactatgccgacagcgtgaagggcaggttcaccctgagccgcgataactccaagaatacactgtatctgcagctgagctccctgcgggacgaggataccggcgtgtactattgcgcccggagattcctggactggtttggcatggacgtgtggggcctgggcaccacagtgacagtgtctagc

SEQ ID NO: 173 - protein, 7 aa, Homo sapiens
GFTFKTY

SEQ ID NO: 174 - protein, 6 aa, Homo sapiens
SGSGTA

SEQ ID NO: 175 - protein, 10 aa, Homo sapiens
RFLDWFGMDV

SEQ ID NO: 176 - protein, 111 aa, Homo sapiens
DIVMTQSPLSLPVTPGEPASISCLSSQSLLQSNGYNYVDWYLQKPGQSPQLLIYLGSNRASGVPDRFSGSGSGTDFTLKISRVEAEDVGVYYCMVTLHPPTFGQGAKVEIK

SEQ ID NO: 177 - DNA, 333 bp, Homo sapiens
  source 1..333: mol_type = genomic DNA
gacatcgtgatgacccagtcccctctgtctctgccagtgacacccggcgagcctgcctctatcagctgtctgagctcccagagcctgctgcagtccaacggctacaattatgtggattggtacctgcagaagccaggccagtccccccagctgctgatctatctgggctctaacagggccagcggcgtgcccgacagattctccggctctggcagcggcaccgacttcaccctgaagatctctcgggtggaggcagaggacgtgggcgtgtactattgcatggtgaccctgcacccacctacattcggccagggagccaaggtggagatcaag

SEQ ID NO: 178 - protein, 16 aa, Homo sapiens
LSSQSLLQSNGYNYVD

SEQ ID NO: 179 - protein, 7 aa, Homo sapiens
LGSNRAS

SEQ ID NO: 180 - protein, 8 aa, Homo sapiens
MVTLHPPT

SEQ ID NO: 181 - protein, 120 aa, Homo sapiens
EGQLVQSGGGLVQPGGSLTLSCEVSGFTFKNYEMNWVRQAPGKGLEWVSYISSGGIAIFHADSVKGRFTVSRDNAKNLLYLQMNSLRVEDTAVYYCARDENNVRRPFDHWGQGTLVTVSS

SEQ ID NO: 182 - DNA, 360 bp, Homo sapiens
  source 1..360: mol_type = genomic DNA
gagggacagctggtgcagtccggcggaggcctggtgcagccaggaggctccctgaccctgtcttgtgaggtgagcggcttcaccttcaagaactacgagatgaattgggtgcggcaggcacctggcaagggcctggagtgggtgtcttatatcagctccggcggaatcgcaatcttccacgcagattccgtgaagggcaggtttaccgtgtctcgcgacaacgccaagaatctgctgtacctgcagatgaacagcctgcgggtggaggacacagccgtgtactattgcgccagggatgagaacaacgtgcggcggcccttcgaccactggggacagggcaccctggtgacagtgtctagc

SEQ ID NO: 183 - protein, 7 aa, Homo sapiens
GFTFKNY

SEQ ID NO: 184 - protein, 6 aa, Homo sapiens
SSGGIA

SEQ ID NO: 185 - protein, 11 aa, Homo sapiens
DENNVRRPFDH

SEQ ID NO: 186 - protein, 109 aa, Homo sapiens
QSVLTQPPSASGSPGQSVTISCTGSSSDVGAYDFVSWFQQYPGQAPKLIIYEVNKRPSGVPARFSGSKSGNTASLTVSGLQAEDEADYFCFSYGGTTNLRVFGGGTKLT

SEQ ID NO: 187 - DNA, 327 bp, Homo sapiens
  source 1..327: mol_type = genomic DNA
cagtctgtgctgacccagccacctagcgcctccggctctcccggccagagcgtgaccatctcctgtacaggcagctcctctgacgtgggcgcctacgatttcgtgagctggtttcagcagtatccaggccaggcccccaagctgatcatctacgaggtgaacaagcggccttccggcgtgccagccagattcagcggctccaagtctggcaataccgcctctctgacagtgagcggcctgcaggcagaggacgaggcagattacttctgcttttcttatggcggcaccacaaacctgcgggtgtttggcggcggcaccaagctgaca

SEQ ID NO: 188 - protein, 14 aa, Homo sapiens
TGSSSDVGAYDFVS

SEQ ID NO: 189 - protein, 7 aa, Homo sapiens
EVNKRPS

SEQ ID NO: 190 - protein, 11 aa, Homo sapiens
FSYGGTTNLRV

SEQ ID NO: 191 - protein, 122 aa, Homo sapiens
EVQLVESGGNLVQPGASLRLSCTASRFNFNKYAMHWVRQTPGKGLEWVSAISWDSTYIDYGNSVKGRFTISRDNTRNSLYLQMNSLTAEDTALYYCAKCEDYLRLCSAYDIWGHGTMVTVSS

SEQ ID NO: 192 - DNA, 366 bp, Homo sapiens
  source 1..366: mol_type = genomic DNA
gaggtgcagctggtggagagcggcggaaacctggtgcagccaggagcctctctgaggctgagctgtaccgcctcccgcttcaactttaataagtacgcaatgcactgggtgcggcagacccctggcaagggcctggagtgggtgtctgccatcagctgggactccacatacatcgattatggcaactccgtgaagggcaggttcaccatctctcgggacaacacaagaaatagcctgtatctgcagatgaattccctgaccgccgaggatacagccctgtactattgcgccaagtgtgaggactacctgcggctgtgctctgcctatgatatctggggccacggcaccatggtgacagtgagctcc

SEQ ID NO: 193 - protein, 7 aa, Homo sapiens
RFNFNKY

SEQ ID NO: 194 - protein, 6 aa, Homo sapiens
SWDSTY

SEQ ID NO: 195 - protein, 13 aa, Homo sapiens
CEDYLRLCSAYDI

SEQ ID NO: 196 - protein, 112 aa, Homo sapiens
DIVMTQSPLSLPVTPGESASISCRSSQSLLHSNGKNYLSWYLQKPGQSPQLLIDLGSNRASGVSDRFSGSGSGTDFTLKISRVEADDVGVYYCMQAVQTPITFGQGTRLAIK

SEQ ID NO: 197 - DNA, 336 bp, Homo sapiens
  source 1..336: mol_type = genomic DNA
gacatcgtgatgacccagtctcctctgagcctgcccgtgacacctggcgagtctgccagcatctcctgtcggagctcccagagcctgctgcactccaacggcaagaattacctgtcttggtatctgcagaagccaggccagagcccccagctgctgatcgatctgggctccaacagggcctccggcgtgtctgacagattctctggcagcggctccggcaccgacttcaccctgaagatcagcagggtggaggccgacgatgtgggcgtgtactattgcatgcaggccgtgcagaccccaatcacattcggccagggaacccgcctggccatcaag

SEQ ID NO: 198 - protein, 16 aa, Homo sapiens
RSSQSLLHSNGKNYLS

SEQ ID NO: 199 - protein, 7 aa, Homo sapiens
LGSNRAS

SEQ ID NO: 200 - protein, 9 aa, Homo sapiens
MQAVQTPIT

SEQ ID NO: 201 - protein, 123 aa, Homo sapiens
QVQLVQSGAELKTPGASVKVSCKASGYTFTGYYIHWVRQAPGEGLEWTGWINPNSGATRYGQKFQGRVTLTSDTSSSTVYMEVSNLTSDDSAVYYCARELSYSIRGTGPLGYWGLGTLVTVSS

SEQ ID NO: 202 - DNA, 369 bp, Homo sapiens
  source 1..369: mol_type = genomic DNA
caggtgcagctggtgcagtccggcgcagagctgaagaccccaggagccagcgtgaaggtgtcctgtaaggcctctggctacaccttcacaggctactatatccactgggtgcggcaggcaccaggagagggcctggagtggaccggctggatcaaccctaatagcggcgccacaagatacggccagaagtttcagggccgcgtgaccctgacaagcgacaccagctcctctacagtgtatatggaggtgtccaacctgacctccgacgattctgccgtgtactattgcgcccgggagctgtcttacagcatcagaggaacaggaccactgggatattggggcctgggcaccctggtgacagtgagctcc

SEQ ID NO: 203 - protein, 7 aa, Homo sapiens
GYTFTGY

SEQ ID NO: 204 - protein, 6 aa, Homo sapiens
NPNSGA

SEQ ID NO: 205 - protein, 14 aa, Homo sapiens
ELSYSIRGTGPLGY

SEQ ID NO: 206 - protein, 108 aa, Homo sapiens
EIVLTQSPGTLSLSPGERATLSCRASQSVASKYLAWYQQKPGQAPRLLIYGASSRATGIPDRFSGSGSGTDFTLTISRLEPEDFAVYYCQYYGSSPLTFGQGTKVEIK

SEQ ID NO: 207 - DNA, 324 bp, Homo sapiens
  source 1..324: mol_type = genomic DNA
gagatcgtgctgacccagtctccaggcacactgtccctgtctccaggagagagggccaccctgtcttgtagagccagccagtccgtggccagcaagtacctggcctggtatcagcagaagccaggacaggcacctaggctgctgatctacggagccagctccagggcaaccggcatccccgaccgcttctctggcagcggctccggcacagacttcaccctgacaatctccaggctggagcctgaggacttcgccgtgtactattgccagtactatggctctagcccactgacctttggccagggcacaaaggtggagatcaag

SEQ ID NO: 208 - protein, 12 aa, Homo sapiens
RASQSVASKYLA

SEQ ID NO: 209 - protein, 7 aa, Homo sapiens
GASSRAT

SEQ ID NO: 210 - protein, 9 aa, Homo sapiens
QYYGSSPLT

SEQ ID NO: 211 - protein, 123 aa, Homo sapiens
EVQLAESGGGVVHPGGSLRLSCTASGFTFSRHSMHWVRQAPGKGLEWVAVISHDGSHKFYVDSVKGRFSISRDNAKNTLYLQMSSLSGADTAVYYCVKDISSRSYGYLAGDSWGQGSLVTVSS

SEQ ID NO: 212 - DNA, 369 bp, Homo sapiens
  source 1..369: mol_type = genomic DNA
gaggtgcagctggccgagtctggcggaggagtggtgcacccaggaggctccctgaggctgtcttgtaccgccagcggcttcacattttctaggcacagcatgcactgggtgcgccaggcacctggcaagggcctggagtgggtggccgtgatctcccacgacggctctcacaagttctacgtggattccgtgaagggccggtttagcatctccagagacaacgccaagaataccctgtatctgcagatgagctccctgtctggcgccgacacagccgtgtactattgcgtgaaggatatctctagcaggagctacggctatctggcaggcgatagctggggacagggctccctggtgaccgtgtcctct

SEQ ID NO: 213 - protein, 7 aa, Homo sapiens
GFTFSRH

SEQ ID NO: 214 - protein, 6 aa, Homo sapiens
SHDGSH

SEQ ID NO: 215 - protein, 14 aa, Homo sapiens
DISSRSYGYLAGDS

SEQ ID NO: 216 - protein, 108 aa, Homo sapiens
DIQMTQSPSSLSASVGDIITITCRASQSVVTYLNWYQQKPGGAPRLLIYTTSKLQSGVPSRFSGSGSGTLFTLTINGLRPEDFATYYCQQSYGTPPFTFGPGTRVEIN

SEQ ID NO: 217 - DNA, 324 bp, Homo sapiens
  source 1..324: mol_type = genomic DNA
gatattcagatgactcagtccccaagcagcctgagcgcctccgtgggcgacatcatcaccatcacatgcagggcctctcagagcgtggtgacctacctgaactggtatcagcagaagccaggaggagcacctaggctgctgatctacaccacatccaagctgcagtctggcgtgccatccagattctccggctctggcagcggcaccctgtttaccctgacaatcaatggcctgcggcccgaggatttcgccacatactattgtcagcagagctatggaacccccccctttacttttggaccaggcacaagagtggagattaac

SEQ ID NO: 218 - protein, 11 aa, Homo sapiens
RASQSVVTYLN

SEQ ID NO: 219 - protein, 7 aa, Homo sapiens
TTSKLQS

SEQ ID NO: 220 - protein, 10 aa, Homo sapiens
QQSYGTPPFT

SEQ ID NO: 221 - protein, 124 aa, Homo sapiens
QVHLQQWGAGLVKPSETLSLTCAVQGGPFSGYYWSWIRQPPGKGLEWIGEINHSGNTHYNPSLKSRVTISVDTSGNYFSLKLTSVTAADAAVYFCARGQQLLRNYYYYSGMDVWGQGTTVTVSS

SEQ ID NO: 222 - DNA, 372 bp, Homo sapiens
  source 1..372: mol_type = genomic DNA
caggtgcacctgcagcagtggggagcaggcctggtgaagccatccgagacactgtctctgacatgtgcagtgcagggaggacccttctctggctactattggagctggatcaggcagccacctggcaagggcctggagtggatcggcgagatcaaccacagcggcaatacccactacaacccctctctgaagagccgggtgaccatcagcgtggacacatccggcaattacttctccctgaagctgacctctgtgacagccgccgatgccgccgtgtatttttgcgcccggggccagcagctgctgagaaactactattactattccggcatggacgtgtggggacagggaaccacagtgacagtgagctcc

SEQ ID NO: 223 - protein, 7 aa, Homo sapiens
GGPFSGY

SEQ ID NO: 224 - protein, 5 aa, Homo sapiens
NHSGN

SEQ ID NO: 225 - protein, 16 aa, Homo sapiens
GQQLLRNYYYYSGMDV

SEQ ID NO: 226 - protein, 107 aa, Homo sapiens
EIVLTQSPGTLSLSPGERATLSCRASQSVTSTYLAWYQQKLGQPPRLLIFGASNRATGIPDRFSGSGSGTDFTLTITRLEPEDFAVYYCQRYGGSITFGQGTRLEIK

SEQ ID NO: 227 - DNA, 321 bp, Homo sapiens
  source 1..321: mol_type = genomic DNA
gagatcgtgctgacacagtccccaggcaccctgagcctgtccccaggagagcgggccacactgtcctgtagagcctctcagagcgtgacctctacatacctggcctggtatcagcagaagctgggccagccccctaggctgctgatcttcggcgcctctaacagggccacaggcatccctgaccgcttctccggctctggcagcggcaccgacttcaccctgacaatcaccagactggagcccgaggacttcgccgtgtactattgccagcggtacggcggcagcatcacatttggccagggcaccagactggagatcaag

SEQ ID NO: 228 - protein, 12 aa, Homo sapiens
RASQSVTSTYLA

SEQ ID NO: 229 - protein, 7 aa, Homo sapiens
GASNRAT

SEQ ID NO: 230 - protein, 8 aa, Homo sapiens
QRYGGSIT

SEQ ID NO: 231 - protein, 126 aa, Homo sapiens
EVQLVQSGGGVVQPRRSLRLSCAASGFTFSNYGMHWVRQVPGKGLQWVAIIWYDGSNKHYAASVQGRFRISRDNSKNTVYLQMDGLRAEDTGMYYCVRDATTATTEGTSQYYFDLWGQGALVTVSS

SEQ ID NO: 232 - DNA, 378 bp, Homo sapiens
  source 1..378: mol_type = genomic DNA
gaggtgcagctggtgcagtccggcggaggagtggtgcagccacggagatctctgaggctgagctgtgccgcctccggcttcaccttttctaactacggaatgcactgggtgcgccaggtgcctggcaagggcctgcagtgggtggccatcatctggtacgacggctccaataagcactatgccgcctctgtgcagggcaggttccgcatctctcgggataacagcaagaataccgtgtatctgcagatggacggcctgcgggccgaggatacaggcatgtactattgcgtgagagacgccaccacagccaccacagagggcaccagccagtactattttgatctgtggggacagggcgccctggtgacagtgagctcc

SEQ ID NO: 233 - protein, 7 aa, Homo sapiens
GFTFSNY

SEQ ID NO: 234 - protein, 6 aa, Homo sapiens
WYDGSN

SEQ ID NO: 235 - protein, 17 aa, Homo sapiens
DATTATTEGTSQYYFDL

SEQ ID NO: 236 - protein, 113 aa, Homo sapiens
DIVMTQSPDSLAVSLGERATINCKSSQTLLYTSNSKNYLAWYQQKVGQPPRLLIYWASTRESGVPDRFSGSGSGTDFTLTISSLLAEDVAVYYCQQYYTTPLTFGGGTKVEVK

SEQ ID NO: 237 - DNA, 339 bp, Homo sapiens
  source 1..339: mol_type = genomic DNA
gacatcgtgatgacccagagccccgattccctggccgtgtctctgggagagagggcaacaatcaactgtaagagctcccagaccctgctgtacacatccaactctaagaattacctggcctggtatcagcagaaagtgggacagccacctaggctgctgatctattgggcctctaccagggagagcggcgtgccagacagattcagcggctccggctctggcacagacttcaccctgacaatctctagcctgctggccgaggacgtggccgtgtactattgccagcagtactataccacacccctgaccttcggcggcggcacaaaggtggaggtgaag

SEQ ID NO: 238 - protein, 17 aa, Homo sapiens
KSSQTLLYTSNSKNYLA

SEQ ID NO: 239 - protein, 7 aa, Homo sapiens
WASTRES

SEQ ID NO: 240 - protein, 9 aa, Homo sapiens
QQYYTTPLT

SEQ ID NO: 241 - protein, 130 aa, Homo sapiens
EVQLVESGGGVVHPGKSLTLSCEASGFTFNDHGIHWVRRAPGKGLEWLALISKDGSKEYSTDSVKGRFTVSRDNSRNTVFLQMKSLTTEDTAIYYCAKDMGQCSSPSCSTMDSYFAMDVWGQGTTVIVSS

SEQ ID NO: 242 - DNA, 390 bp, Homo sapiens
  source 1..390: mol_type = genomic DNA
gaggtgcagctggtggagtccggcggaggagtggtgcaccctggcaagtctctgaccctgagctgtgaggccagcggcttcaccttcaacgaccacggcatccactgggtgcggagagcacctggcaagggcctggagtggctggccctgatctctaaggacggcagcaaggagtacagcaccgattccgtgaagggccggttcacagtgtccagggataactctcgcaataccgtgtttctgcagatgaagtctctgaccacagaggacacagccatctactattgcgccaaggatatgggccagtgcagctccccctcctgttctaccatggacagctatttcgcaatggacgtgtggggacagggaaccacagtgatcgtgtctagc

SEQ ID NO: 243 - protein, 7 aa, Homo sapiens
GFTFNDH

SEQ ID NO: 244 - protein, 6 aa, Homo sapiens
SKDGSK

SEQ ID NO: 245 - protein, 21 aa, Homo sapiens
DMGQCSSPSCSTMDSYFAMDV

SEQ ID NO: 246 - protein, 113 aa, Homo sapiens
DIVMTQSPLSLPVTPGEPASISCRSSQNLRHNNGYNYLNWYLQKPGQSPQLLIYLGSIRASGVPDRFSGSGSGTDFTLKISRVEAEDVGVYYCMQALQTPPWTFGQGTKVDFK

SEQ ID NO: 247 - DNA, 339 bp, Homo sapiens
  source 1..339: mol_type = genomic DNA
gacatcgtgatgacccagtcccctctgtctctgccagtgacacccggcgagcctgcctctatcagctgtcggagctcccagaacctgagacacaacaatggctacaactatctgaattggtacctgcagaagccaggccagtctccccagctgctgatctatctgggcagcatcagggcctccggcgtgcccgaccgcttctccggctctggcagcggcaccgacttcaccctgaagatcagccgggtggaggcagaggacgtgggcgtgtactattgcatgcaggccctgcagacccccccttggacattcggccagggcaccaaggtggacttcaag

SEQ ID NO: 248 - protein, 16 aa, Homo sapiens
RSSQNLRHNNGYNYLN

SEQ ID NO: 249 - protein, 7 aa, Homo sapiens
LGSIRAS

SEQ ID NO: 250 - protein, 10 aa, Homo sapiens
MQALQTPPWT

SEQ ID NO: 251 - protein, 118 aa, Homo sapiens
QVQLVQSGAEVKKPGASVKVSCKASGYTFTSHYMHWVRQAPGQGLEWMGIISPTGDFTNYAQKFQGRVTLTRDTSTSTDYMEVTSLRSEDTAVYYCARDCSAWAPDYWGQGTLVTVSS

SEQ ID NO: 252 - DNA, 354 bp, Homo sapiens
  source 1..354: mol_type = genomic DNA
caggtgcagctggtgcagtccggcgcagaggtgaagaagccaggagccagcgtgaaggtgtcctgtaaggcctctggctacaccttcacatctcactatatgcactgggtgcggcaggcaccaggacagggcctggagtggatgggcatcatcagccctacaggcgacttcaccaactacgcccagaagtttcagggccgggtgaccctgacaagagacacctctacaagcaccgattatatggaggtgacatccctgaggtctgaggataccgccgtgtactattgcgcaagggactgttccgcctgggcccccgattactggggacagggcacactggtgaccgtgagctcc

SEQ ID NO: 253 - protein, 7 aa, Homo sapiens
GYTFTSH

SEQ ID NO: 254 - protein, 6 aa, Homo sapiens
SPTGDF

SEQ ID NO: 255 - protein, 9 aa, Homo sapiens
DCSAWAPDY

SEQ ID NO: 256 - protein, 108 aa, Homo sapiens
QSALTRPPSVSRCPGQSITISCSGTSSDVGHDNHVSWYQQHPGRAPKLMVYEVRNRPSGVSDRFSGSKSGNTASLTISGLQAEDEATYYCCSYTTTHRYIFGGGTKLT

SEQ ID NO: 257 - DNA, 324 bp, Homo sapiens
  source 1..324: mol_type = genomic DNA
cagtctgccctgacaaggcccccttctgtgagccgctgccctggacagagcatcacaatctcctgttctggcaccagctccgacgtgggccacgataaccacgtgtcctggtaccagcagcacccaggaagggcacccaagctgatggtgtatgaggtgcggaacagaccaagcggcgtgtccgacaggttcagcggctccaagtctggcaatacagcctctctgaccatcagcggcctgcaggcagaggatgaggcaacctactattgctgttcttacaccacaacccaccggtatatctttggcggcggcacaaagctgacc

SEQ ID NO: 258 - protein, 14 aa, Homo sapiens
SGTSSDVGHDNHVS

SEQ ID NO: 259 - protein, 7 aa, Homo sapiens
EVRNRPS

SEQ ID NO: 260 - protein, 10 aa, Homo sapiens
CSYTTTHRYI

SEQ ID NO: 261 - protein, 123 aa, Homo sapiens
QVQLLGSGPGLVKPSETLSLTCTVSGASISSPGYYWGFIRQSPGKGLEWIGSMVSGGTTYYNPSLKSRVTISMDMSNNQFSLRLNSVTAADTALYYCARGSRQLVRRATIDYWGQGALFTVSP

SEQ ID NO: 262 - DNA, 369 bp, Homo sapiens
  source 1..369: mol_type = genomic DNA
caggtgcagctgctgggcagcggcccaggcctggtgaagccttctgagacactgagcctgacctgtacagtgtctggcgccagcatcagctccccaggctactattggggcttcatcaggcagagcccaggcaagggcctggagtggatcggctccatggtgtctggcggcaccacatactataaccctagcctgaagtcccgggtgacaatctccatggacatgtctaacaatcagttcagcctgaggctgaattccgtgaccgccgccgatacagccctgtactattgcgcaaggggctcccgccagctggtgcggagagcaaccatcgactactggggacagggcgccctgtttacagtgtctccc

SEQ ID NO: 263 - protein, 9 aa, Homo sapiens
GASISSPGY

SEQ ID NO: 264 - protein, 5 aa, Homo sapiens
VSGGT

SEQ ID NO: 265 - protein, 13 aa, Homo sapiens
GSRQLVRRATIDY

SEQ ID NO: 266 - protein, 108 aa, Homo sapiens
QSVLTGPPSVSAGPGQQVFISCSGNSSNIGNNYVSWYQQLPGTAPKLLIYDSNKRPSGIPDRFSGSKSGTSATLGITGLQTGDEADYYCGTWDSSLSAGVFGGGTKLT

SEQ ID NO: 267 - DNA, 324 bp, Homo sapiens
  source 1..324: mol_type = genomic DNA
cagtctgtgctgaccggaccaccttccgtgtctgccggaccaggacagcaggtgttcatcagctgttccggcaacagctccaatatcggcaacaattacgtgtcttggtatcagcagctgccaggcacagcccccaagctgctgatctacgactctaacaagcggcctagcggcatcccagatagattctctggcagcaagtccggcaccagcgccacactgggcatcaccggcctgcagacaggcgacgaggcagattactattgcggaacctgggactctagcctgtccgccggcgtgtttggaggaggaaccaagctgaca

SEQ ID NO: 268 - protein, 13 aa, Homo sapiens
SGNSSNIGNNYVS

SEQ ID NO: 269 - protein, 7 aa, Homo sapiens
DSNKRPS

SEQ ID NO: 270 - protein, 11 aa, Homo sapiens
GTWDSSLSAGV

SEQ ID NO: 271 - protein, 124 aa, Homo sapiens
EVQLVESGGGLVKPGESLRLSCAASGFTFSSYSMSWVRQAPGKGLEWVSCITSSGHTYYADSVKGRFAISRDNGKNSLYLQMNNLRAEDTAVYFCAKELGAHSGLFYNGVFDYWGQGNPVTVSS

SEQ ID NO: 272 - DNA, 372 bp, Homo sapiens
  source 1..372: mol_type = genomic DNA
gaggtgcagctggtggagtccggcggaggcctggtgaagccaggcgagtctctgaggctgagctgtgccgcctccggcttcacctttagctcctacagcatgtcctgggtgcgccaggcacctggcaagggcctggagtgggtgtcctgcatcacctctagcggccacacatactatgccgactctgtgaagggccggttcgccatcagccgggataacggcaagaatagcctgtacctgcagatgaacaatctgcgggccgaggacaccgccgtgtatttttgtgcaaaggagctgggagcacactctggcctgttctacaacggcgtgtttgattattggggccagggcaatcccgtgacagtgtcctct

SEQ ID NO: 273 - protein, 7 aa, Homo sapiens
GFTFSSY

SEQ ID NO: 274 - protein, 5 aa, Homo sapiens
TSSGH

SEQ ID NO: 275 - protein, 16 aa, Homo sapiens
ELGAHSGLFYNGVFDY

SEQ ID NO: 276 - protein, 108 aa, Homo sapiens
QSALTQPASVSGSPGQSITISCTGTSSDVGGYNYVSWYQQHPGKAPKLMIYEVSNRPSGVSNRFSGSKGNTASLTISGLRGEDEADYYCSSYTSSSTLVVFGGGTKLT

SEQ ID NO: 277 - DNA, 324 bp, Homo sapiens
  source 1..324: mol_type = genomic DNA
cagtccgccctgacccagccagcctccgtgtctggcagccccggccagtctatcacaatcagctgtaccggcacaagctccgacgtgggcggctacaactacgtgagctggtaccagcagcacccaggcaaggcacctaagctgatgatctatgaggtgtccaacaggccaagcggcgtgtccaatagattctccggctctaagggcaataccgcctccctgacaatctctggcctgaggggagaggacgaggcagattactattgctctagctacacctcctctagcacactggtggtgtttggcggcggcaccaagctgaca

SEQ ID NO: 278 - protein, 14 aa, Homo sapiens
TGTSSDVGGYNYVS

SEQ ID NO: 279 - protein, 7 aa, Homo sapiens
EVSNRPS

SEQ ID NO: 280 - protein, 11 aa, Homo sapiens
SSYTSSSTLVV

SEQ ID NO: 281 - protein, 124 aa, Homo sapiens; identical to SEQ ID NO: 221

SEQ ID NO: 282 - DNA, 372 bp, Homo sapiens; identical to SEQ ID NO: 222
  source 1..372: mol_type = genomic DNA

SEQ ID NO: 283 - protein, 7 aa, Homo sapiens
GGPFSGY

SEQ ID NO: 284 - protein, 5 aa, Homo sapiens
NHSGN

SEQ ID NO: 285 - protein, 16 aa, Homo sapiens
GQQLLRNYYYYSGMDV

SEQ ID NO: 286 - protein, 108 aa, Homo sapiens
QSALTQPASVSGSPGQSITISCTETSRDVGDYNYVSWYQQHPGPAPKLIMYEVHKRPSGISNRFSGSKSGTTASLTISGLQADDEGDYYCSSYTDKNTYVFGSGTQVT

SEQ ID NO: 287 - DNA, 324 bp, Homo sapiens
  source 1..324: mol_type = genomic DNA
cagtctgccctgacccagccagcctctgtgagcggctcccctggccagtccatcacaatctcttgtaccgagacatctcgggacgtgggcgattacaactatgtgagctggtaccagcagcacccaggacctgcaccaaagctgatcatgtatgaggtgcacaagcggccctctggcatcagcaatagattctctggcagcaagtccggcaccacagccagcctgaccatctccggcctgcaggcagacgatgagggcgactactattgcagctcctacaccgataagaacacatacgtgttcggcagcggcacccaggtgaca

SEQ ID NO: 288 - protein, 14 aa, Homo sapiens
TETSRDVGDYNYVS

SEQ ID NO: 289 - protein, 7 aa, Homo sapiens
EVHKRPS

SEQ ID NO: 290 - protein, 10 aa, Homo sapiens
SSYTDKNTYV

SEQ ID NO: 291 - protein, 447 aa, Homo sapiens
EAALLVCQYTIQSLIHLTGEDPGFFNVEIPEFPFYPTCNVCTADVNVTINFDVGGKKHQLDLDFGQLTPHTKAVYQPRGAFGGSENATNLFLLELLGAGELALTMRSKKLPINVTTGEEQQVSLESVDVYFQDVFGTMWCHHAEMQNPVYLIPETVPYIDWDNCNSTNITAVVRAQGLDVTLPLSLPTSAQDSNFSVKTEMLGNEIDIECIMEDGEISQVLPGDNKFNITCSGYESHVPSGGILTSTSPVATPIPGTGYAYSLRLTPRPVSRFLGNNSILYVFYSGNGPKASGGRYCIQSNIVFSDEIPASQDMPTNTTDITYVGDNATYSVPMVTSEDANSPNVTVTAFWAWPNNTETDFKCKWTLTSGTPSGCENISGAFASNRTFDITVSGLGTAPKTLIITRTATNATTTTHKVIFSKAPGSGLNDIFEAQKIEWHEHHHHHH

SEQ ID NO: 292 - DNA, 1341 bp, Homo sapiens
  source 1..1341: mol_type = genomic DNA
gaagctgccctgctcgtgtgccagtacaccatccagagcctgatccacctgaccggcgaggaccccggcttcttcaacgtggaaatccccgagttccccttctaccctacctgcaacgtgtgcaccgccgacgtgaacgtgaccatcaacttcgacgtgggcggcaagaagcaccagctggacctggatttcggccagctgacccctcacaccaaggccgtgtatcagcccagaggcgcctttggcggcagcgagaacgccaccaatctgtttctgctggaactcctaggcgccggcgagctggccctgaccatgagaagcaagaaactgcccatcaatgtgaccacaggcgaggaacagcaggtgtccctggaaagcgtggacgtgtactttcaagacgtgttcggcaccatgtggtgccaccacgccgagatgcagaaccccgtgtacctgatccccgagacagtgccctacatcgattgggacaactgcaacagcaccaacatcaccgccgtcgtgcgggcccagggactggatgtgacactgcctctgagcctgcctaccagcgcccaggacagcaacttcagcgtgaaaaccgagatgctgggcaacgagatcgacatcgagtgcatcatggaagatggcgagatcagccaggtgctgcccggcgacaacaagttcaacatcacatgcagcggctacgagagccacgtgccatctggcggcatcctgaccagcacaagcccagtggccacacccatccctggcacaggctacgcctacagcctgagactgacccccagacccgtgtccagattcctgggcaacaacagcatcctgtacgtgttctacagcggcaacggccccaaggcctctggcggccggtactgtatccagagcaacatcgtgttcagcgacgagatccccgccagccaggacatgcccaccaataccaccgacatcacgtacgtgggcgacaatgccacctacagcgtgccaatggtcacctccgaggacgccaacagccccaacgtgaccgtgacagccttttgggcctggcctaacaacaccgagacagacttcaagtgcaagtggaccctgacctccggcacccctagcggctgcgagaatatcagcggagccttcgccagcaaccggaccttcgatatcaccgtgtctggcctgggcaccgcccccaagaccctgatcatcaccagaaccgccacaaatgccaccaccacaacccacaaagtgatcttcagcaaggcccccggctctggcctgaacgacatttttgaggcccagaagattgagtggcatgaacatcaccaccaccaccat

SEQ ID NO: 293 - DNA, 5118 bp, Homo sapiens
  source 1..5118: mol_type = genomic DNA
tcgcgcgtttcggtgatgacggtgaaaacctctgacacatgcagctcccggagacggtcacagcttgtctgtaagcggatgccgggagcagacaagcccgtcagggcgcgtcagcgggtgttggcgggtgtcggggctggcttaactatgcggcatcagagcagattgtactgagagtgcaccatatgcggtgtgaaataccgcacagatgcgtaaggagaaaataccgcatcagattggctattggccattgcatacgttgtatccatatcataatatgtacatttatattggctcatgtccaacattaccgccatgttgacattgattattgactagttattaatagtaatcaattacggggtcattagttcatagcccatatatggagttccgcgttacataacttacggtaaatggcccgcctggctgaccgcccaacgacccccgcccattgacgtcaataatgacgtatgttcccatagtaacgccaatagggactttccattgacgtcaatgggtggagtatttacggtaaactgcccacttggcagtacatcaagtgtatcatatgccaagtacgccccctattgacgtcaatgacggtaaatggcccgcctggcattatgcccagtacatgaccttatgggactttcctacttggcagtacatctacgtattagtcatcgctattaccatggtgatgcggttttggcagtacatcaatgggcgtggatagcggtttgactcacggggatttccaagtctccaccccattgacgtcaatgggagtttgttttggcaccaaaatcaacgggactttccaaaatgtcgtaacaactccgccccattgacgcaaatgggcggtaggcgtgtacggtgggaggtctatataagcagagctcgtttagtgaaccgtcagatcgcctggagacgccatccacgctgttttgacctccatagaagacaccgggaccgatccagcctccatcggctcgcatctctccttcacgcgcccgccgccctacctgaggccgccatccacgccggttgagtcgcgttctgccgcctcccgcctgtggtgcctcctgaactgcgtccgccgtctaggtaagtttaaagctcaggtcgagaccgggcctttgtccggcgctcccttggagcctacctagactcagccggctctccacgctttgcctgaccctgcttgctcaactctagttaacggtggagggcagtgtagtctgagcagtacacgttgctgccgcgcgcgccaccagacataatagctgacagactaacagactgttcctttccatgggtcttttctgcagtcaccgtcgtcgacacgtgtgatcagatatcgcggccgctctagaccaccatgggatggtcatgtatcatcctttttctagtagcaactgcaaccggtgtacattcccagtctgccctgactcagcctccctctgtgtctgggtctcctggacagtcggtcaccatctcctgcactggaaccagcagtgacgttgatggttataactatgtctcctggtaccaacaacatccaggcaaagcccccaaactcatgatttatggtgtcagcaatcggccctcaggggtctctgatcgcttctctggctccaagtctggcaacacggcctccctgaccatctctgggctccaggctgaggacgaggctgattattactgttgttcatctacaaccagttacacttacatcttcggaactgggaccaaggtcacagtactaggtcagcccaaggctgccccctcggtcactctcttcccgccctcctctgaggagcttcaagccaacaaggccacactagtgtgtctgatcagtgacttctacccgggagccgtggaagtggcctggaaggcagatggcagcgctgtcaacgcgggagtggagaccaccaaaccctccaaacagagcaacaacaagtacgcggccagcagctacctgagcctgacgtccgaccagtggaagtcccacaagagctacagctgccaggtcacgcacgaagggagcaccgtggagaagacagtggcccctgcagaatgttcatagggatccagatctgctgtgccttctagttgccagccatctgttgtttgcccctcccccgtgccttccttgaccctggaaggtgccactcccactgtcctttcctaataaaatgaggaaattgcatcgcattgtctgagtaggtgtcattctattctggggggtggggtggggcaggacagcaagggggaggattgggaagacaatagcaggcatgctggggatgcggtgggctctatgggtacccaggtgctgaagaattgacccggttcctcctgggccagaaagaagcaggcacatccccttctctgtgacacaccctgtccacgcccctggttcttagttccagccccactcataggacactcatagctcaggagggctccgccttcaatcccacccgctaaagtacatggagcggtctctccctccctcatcagcccaccaaaccaaacctagcctccaagagtgggaagaaattaaagcaagataggctattaagtgcagagggagagaaaatgcctccaacatgtgaggaagtaatgagagaaatcatagaattttaaggccatgatttaaggccatcatggccttaatcttccgcttcctcgctcactgactcgctgcgctcggtcgttcggctgcggcgagcggtatcagctcactcaaaggcggtaatacggttatccacagaatcaggggataacgcaggaaagaacatgtgagcaaaaggccagcaaaaggccaggaaccgtaaaaaggccgcgttgctggcgtttttccataggctccgcccccctgacgagcatcacaaaaatcgacgctcaagtcagaggtggcgaaacccgacaggactataaagataccaggcgtttccccctggaagctccctcgtgcgctctcctgttccgaccctgccgcttaccggatacctgtccgcctttctcccttcgggaagcgtggcgctttctcatagctcacgctgtaggtatctcagttcggtgtaggtcgttcgctccaagctgggctgtgtgcacgaaccccccgttcagcccgaccgctgcgccttatccggtaactatcgtcttgagtccaacccggtaagacacgacttatcgccactggcagcagccactggtaacaggattagcagagcgaggtatgtaggcggtgctacagagttcttgaagtggtggcctaactacggctacactagaagaacagtatttggtatctgcgctctgctgaagccagttaccttcggaaaaagagttggtagctcttgatccggcaaacaaaccaccgctggtagcggtggtttttttgtttgcaagcagcagattacgcgcagaaaaaaaggatctcaagaagatcctttgatcttttctacggggtctgacgctcagtggaacgaaaactcacgttaagggattttggtcatgagattatcaaaaaggatcttcacctagatccttttaaattaaaaatgaagttttaaatcaatctaaagtatatatgagtaaacttggtctgacagttaccaatgcttaatcagtgaggcacctatctcagcgatctgtctatttcgttcatccatagttgcctgactcggggggggggggcgctgaggtctgcctcgtgaagaaggtgttgctgactcataccaggcctgaatcgccccatcatccagccagaaagtgagggagccacggttgatgagagctttgttgtaggtggaccagttggtgattttgaacttttgctttgccacggaacggtctgcgttgtcgggaagatgcgtgatctgatccttcaactcagcaaaagttcgatttattcaacaaagccgccgtcccgtcaagtcagcgtaatgctctgccagtgttacaaccaattaaccaattctgattagaaaaactcatcgagcatcaaatgaaactgcaatttattcatatcaggattatcaataccatatttttgaaaaagccgtttctgtaatgaaggagaaaactcaccgaggcagttccataggatggcaagatcctggtatcggtctgcgattccgactcgtccaacatcaatacaacctattaatttcccctcgtcaaaaataaggttatcaagtgagaaatcaccatgagtgacgactgaatccggtgagaatggcaaaagcttatgcatttctttccagacttgttcaacaggccagccattacgctcgtcatcaaaatcactcgcatcaaccaaaccgttattcattcgtgattgcgcctgagcgagacgaaatacgcgatcgctgttaaaaggacaattacaaacaggaatcgaatgcaaccggcgcaggaacactgccagcgcatcaacaatattttcacctgaatcaggatattcttctaatacctggaatgctgttttcccggggatcgcagtggtgagtaaccatgcatcatcaggagtacggataaaatgcttgatggtcggaagaggcataaattccgtcagccagtttagtctgaccatctcatctgtaacatcattggcaacgctacctttgccatgtttcagaaacaactctggcgcatcgggcttcccatacaatcgatagattgtcgcacctgattgcccgacattatcgcgagcccatttatacccatataaatcagcatccatgttggaatttaatcgcggcctcgagcaagacgtttcccgttgaatatggctcataacaccccttgtattactgtttatgtaagcagacagttttattgttcatgatgatatatttttatcttgtgcaatgtaacatcagagattttgagacacaacgtggctttccccccccccccattattgaagcatttatcagggttattgtctcatgagcggatacatatttgaatgtatttagaaaaataaacaaataggggttccgcgcacatttccccgaaaagtgccacctgacgtctaagaaaccattattatcatgacattaacctataaaaataggcgtatcacgaggccctttcgtc